European Patent Application EP 4 328 306 A2, published February 28, 2024. Title: ANGELMAN SYNDROME ANTISENSE TREATMENT. Applicant: The Texas A&M University System. Application EP. The sequence listing filed with the application follows.

SEQUENCE LISTING (605 sequences)

SEQ ID NO: 1 - DNA, 184 bp, synthetic construct
  misc_feature 1..184: note = Synthetic Construct
  source 1..184: mol_type = other DNA
atgatgatatggaagaaaagcactctttggcctgttgtgactgggacagttgacagcacccaggtgtcctttaatgaaaatgctcttgacaccaatgcatcctagcatcacagcttcaggaagccttctcaagtgtgcatggggagtactatgtctttcatcaataatgaaatcttctgatttg

SEQ ID NO: 2 - DNA, 133 bp, synthetic construct
  misc_feature 1..133: note = Synthetic Construct
  source 1..133: mol_type = other DNA
taagacatgctgccaagagatgtgccattctattataaaagatcagtagcttcctttaccgacgtgtatattctatctagaacattgagctatggaagactcccacctaagggaattagttttacaccttcag

SEQ ID NO: 3 - DNA, 125 bp, synthetic construct
  misc_feature 1..125: note = Synthetic Construct
  source 1..125: mol_type = other DNA
ataaagactgctgagaagagcaccctctggtgttgtcacagaggcaagtgctaccgcacaggcatgctgcagtgaatttaactgatcctctgtccctgcaaccgttgtttaaggatgctattctg

SEQ ID NO: 4 - DNA, 129 bp, synthetic construct
  misc_feature 1..129: note = Synthetic Construct
  source 1..129: mol_type = other DNA
aaaagactgtggaggaagaaaaccctttaccctgttgttcagggagaaactgacaccactcaactgcctggcactgaaaatgtggcatccagtccactttaccatcagtgtttaaggaaaccatctctg

SEQ ID NO: 5 - DNA, 117 bp, synthetic construct
  misc_feature 1..117: note = Synthetic Construct
  source 1..117: mol_type = other DNA
ataaggatgactgaggaagagtactctttggcttgttgacaccagcacagctgacacacccagatatctgtttggtctcctgtgaactttcaaccaggatttaaggatgccactctg

SEQ ID NO: 6 - DNA, 20 bp, synthetic construct
  misc_feature 1..20: note = Synthetic Construct
  source 1..20: mol_type = other DNA
tagaggtgaaggccaggcac

SEQ ID NO: 7 - DNA, 20 bp, synthetic construct
  misc_feature 1..20: note = Synthetic Construct
  source 1..20: mol_type = other DNA
gtactcttcctcagtcatcc

SEQ ID NO: 8 - DNA, 20 bp, synthetic construct
  misc_feature 1..20: note = Synthetic Construct
  source 1..20: mol_type = other DNA
tgtcagtttctccctgaaca

SEQ ID NO: 9 - DNA, 20 bp, synthetic construct
  misc_feature 1..20: note = Synthetic Construct
  source 1..20: mol_type = other DNA
tagaatggcacatctcttgg

SEQ ID NO: 10 - DNA, 20 bp, synthetic construct
  misc_feature 1..20: note = Synthetic Construct
  source 1..20: mol_type = other DNA
gttttcttcctccacagtct

SEQ ID NO: 11 - DNA, 20 bp, synthetic construct
  misc_feature 1..20: note = Synthetic Construct
  source 1..20: mol_type = other DNA
ctggtgtcaacaagccaaag

SEQ ID NO: 12 - RNA, 18 nt, synthetic construct
  misc_feature 1..18: note = Synthetic Construct
  source 1..18: mol_type = other RNA
gaaaatgctcttgacacc

SEQ ID NO: 13 - RNA, 19 nt, synthetic construct
  misc_feature 1..19: note = Synthetic Construct
  source 1..19: mol_type = other RNA
gaaaatgctcttgacacca

SEQ ID NO: 14 - RNA, 20 nt, synthetic construct
  misc_feature 1..20: note = Synthetic Construct
  source 1..20: mol_type = other RNA
gaaaatgctcttgacaccaa

SEQ ID NO: 15 - DNA, 18 bp, synthetic construct
  misc_feature 1..18: note = Synthetic Construct
  source 1..18: mol_type = other DNA
ggtgtcaagagcattttc

SEQ ID NO: 16 - DNA, 19 bp, synthetic construct
  misc_feature 1..19: note = Synthetic Construct
  source 1..19: mol_type = other DNA
tggtgtcaagagcattttc

SEQ ID NO: 17 - DNA, 20 bp, synthetic construct
  misc_feature 1..20: note = Synthetic Construct
  source 1..20: mol_type = other DNA
ttggtgtcaagagcattttc

SEQ ID NO: 18 - RNA, 18 nt, synthetic construct
  misc_feature 1..18: note = Synthetic Construct
  source 1..18: mol_type = other RNA
catgctgccaagagatgt

SEQ ID NO: 19 - RNA, 19 nt, synthetic construct
  misc_feature 1..19: note = Synthetic Construct
  source 1..19: mol_type = other RNA
catgctgccaagagatgtg

SEQ ID NO: 20 - RNA, 20 nt, synthetic construct
  misc_feature 1..20: note = Synthetic Construct
  source 1..20: mol_type = other RNA
catgctgccaagagatgtgc

SEQ ID NO: 21 - RNA, 18 nt, synthetic construct
  misc_feature 1..18: note = Synthetic Construct
  source 1..18: mol_type = other RNA
atgctgccaagagatgtg

SEQ ID NO: 22 - RNA, 19 nt, synthetic construct
  misc_feature 1..19: note = Synthetic Construct
  source 1..19: mol_type = other RNA
atgctgccaagagatgtgc

SEQ ID NO: 23 - RNA, 20 nt, synthetic construct
  misc_feature 1..20: note = Synthetic Construct
  source 1..20: mol_type = other RNA
atgctgccaagagatgtgcc

SEQ ID NO: 24 - RNA, 19 nt, synthetic construct
  misc_feature 1..19: note = Synthetic Construct
  source 1..19: mol_type = other RNA
tgctgccaagagatgtgcc

SEQ ID NO: 25 - RNA, 20 nt, synthetic construct
  misc_feature 1..20: note = Synthetic Construct
  source 1..20: mol_type = other RNA
tgctgccaagagatgtgcca

SEQ ID NO: 26 - RNA, 19 nt, synthetic construct
  misc_feature 1..19: note = Synthetic Construct
  source 1..19: mol_type = other RNA
gctgccaagagatgtgcca

SEQ ID NO: 27 - RNA, 20 nt, synthetic construct
  misc_feature 1..20: note = Synthetic Construct
  source 1..20: mol_type = other RNA
gctgccaagagatgtgccat

SEQ ID NO: 28 - RNA, 18 nt, synthetic construct
  misc_feature 1..18: note = Synthetic Construct
  source 1..18: mol_type = other RNA
ctgccaagagatgtgcca

SEQ ID NO: 29 - RNA, 19 nt, synthetic construct
  misc_feature 1..19: note = Synthetic Construct
  source 1..19: mol_type = other RNA
ctgccaagagatgtgccat

SEQ ID NO: 30 - RNA, 20 nt, synthetic construct
  misc_feature 1..20: note = Synthetic Construct
  source 1..20: mol_type = other RNA
ctgccaagagatgtgccatt

SEQ ID NO: 31 - RNA, 18 nt, synthetic construct
  misc_feature 1..18: note = Synthetic Construct
  source 1..18: mol_type = other RNA
tgccaagagatgtgccat

SEQ ID NO: 32 - RNA, 19 nt, synthetic construct
  misc_feature 1..19: note = Synthetic Construct
  source 1..19: mol_type = other RNA
tgccaagagatgtgccatt

SEQ ID NO: 33 - RNA, 20 nt, synthetic construct
  misc_feature 1..20: note = Synthetic Construct
  source 1..20: mol_type = other RNA
tgccaagagatgtgccattc

SEQ ID NO: 34 - RNA, 18 nt, synthetic construct
  misc_feature 1..18: note = Synthetic Construct
  source 1..18: mol_type = other RNA
gccaagagatgtgccatt

SEQ ID NO: 35 - RNA, 19 nt, synthetic construct
  misc_feature 1..19: note = Synthetic Construct
  source 1..19: mol_type = other RNA
gccaagagatgtgccattc

SEQ ID NO: 36 - RNA, 20 nt, synthetic construct
  misc_feature 1..20: note = Synthetic Construct
  source 1..20: mol_type = other RNA
gccaagagatgtgccattct

SEQ ID NO: 37 - RNA, 18 nt, synthetic construct
  misc_feature 1..18: note = Synthetic Construct
  source 1..18: mol_type = other RNA
ccaagagatgtgccattc

SEQ ID NO: 38 - RNA, 19 nt, synthetic construct
  misc_feature 1..19: note = Synthetic Construct
  source 1..19: mol_type = other RNA
ccaagagatgtgccattct

SEQ ID NO: 39 - RNA, 20 nt, synthetic construct
  misc_feature 1..20: note = Synthetic Construct
  source 1..20: mol_type = other RNA
ccaagagatgtgccattcta

SEQ ID NO: 40 - RNA, 18 nt, synthetic construct
  misc_feature 1..18: note = Synthetic Construct
  source 1..18: mol_type = other RNA
caagagatgtgccattct

SEQ ID NO: 41 - RNA, 19 nt, synthetic construct
  misc_feature 1..19: note = Synthetic Construct
  source 1..19: mol_type = other RNA
caagagatgtgccattcta

SEQ ID NO: 42 - RNA, 20 nt, synthetic construct
  misc_feature 1..20: note = Synthetic Construct
  source 1..20: mol_type = other RNA
caagagatgtgccattctat

SEQ ID NO: 43 - RNA, 18 nt, synthetic construct
  misc_feature 1..18: note = Synthetic Construct
  source 1..18: mol_type = other RNA
tcctttaccgacgtgtat

SEQ ID NO: 44 - RNA, 19 nt, synthetic construct
  misc_feature 1..19: note = Synthetic Construct
  source 1..19: mol_type = other RNA
tcctttaccgacgtgtata

SEQ ID NO: 45 - RNA, 20 nt, synthetic construct
  misc_feature 1..20: note = Synthetic Construct
  source 1..20: mol_type = other RNA
tcctttaccgacgtgtatat

SEQ ID NO: 46 - RNA, 18 nt, synthetic construct
  misc_feature 1..18: note = Synthetic Construct
  source 1..18: mol_type = other RNA
cctttaccgacgtgtata

SEQ ID NO: 47 - RNA, 19 nt, synthetic construct
  misc_feature 1..19: note = Synthetic Construct
  source 1..19: mol_type = other RNA
cctttaccgacgtgtatat

SEQ ID NO: 48 - RNA, 20 nt, synthetic construct
  misc_feature 1..20: note = Synthetic Construct
  source 1..20: mol_type = other RNA
cctttaccgacgtgtatatt

SEQ ID NO: 49 - RNA, 20 nt, synthetic construct
  misc_feature 1..20: note = Synthetic Construct
  source 1..20: mol_type = other RNA
accgacgtgtatattctatc

SEQ ID NO: 50 - RNA, 19 nt, synthetic construct
  misc_feature 1..19: note = Synthetic Construct
  source 1..19: mol_type = other RNA
ccgacgtgtatattctatc

SEQ ID NO: 51 - RNA, 20 nt, synthetic construct
  misc_feature 1..20: note = Synthetic Construct
  source 1..20: mol_type = other RNA
ccgacgtgtatattctatct

SEQ ID NO: 52 - RNA, 20 nt, synthetic construct
  misc_feature 1..20: note = Synthetic Construct
  source 1..20: mol_type = other RNA
tctagaacattgagctatgg

SEQ ID NO: 53 - RNA, 18 nt, synthetic construct
  misc_feature 1..18: note = Synthetic Construct
  source 1..18: mol_type = other RNA
cattgagctatggaagac

SEQ ID NO: 54 - RNA, 20 nt, synthetic construct
  misc_feature 1..20: note = Synthetic Construct
  source 1..20: mol_type = other RNA
ctatggaagactcccaccta

SEQ ID NO: 55 - RNA, 19 nt, synthetic construct
  misc_feature 1..19: note = Synthetic Construct
  source 1..19: mol_type = other RNA
tatggaagactcccaccta

SEQ ID NO: 56 - RNA, 20 nt, synthetic construct
  misc_feature 1..20: note = Synthetic Construct
  source 1..20: mol_type = other RNA
tatggaagactcccacctaa

SEQ ID NO: 57 - RNA, 18 nt, synthetic construct
  misc_feature 1..18: note = Synthetic Construct
  source 1..18: mol_type = other RNA
atggaagactcccaccta

SEQ ID NO: 58 - RNA, 19 nt, synthetic construct
  misc_feature 1..19: note = Synthetic Construct
  source 1..19: mol_type = other RNA
atggaagactcccacctaa

SEQ ID NO: 59 - RNA, 18 nt, synthetic construct
  misc_feature 1..18: note = Synthetic Construct
  source 1..18: mol_type = other RNA
tggaagactcccacctaa

SEQ ID NO: 60 - RNA, 20 nt, synthetic construct
  misc_feature 1..20: note = Synthetic Construct
  source 1..20: mol_type = other RNA
gactcccacctaagggaatt

SEQ ID NO: 61 - RNA, 18 nt, synthetic construct
  misc_feature 1..18: note = Synthetic Construct
  source 1..18: mol_type = other RNA
actcccacctaagggaat

SEQ ID NO: 62 - RNA, 19 nt, synthetic construct
  misc_feature 1..19: note = Synthetic Construct
  source 1..19: mol_type = other RNA
actcccacctaagggaatt

SEQ ID NO: 63 - RNA, 20 nt, synthetic construct
  misc_feature 1..20: note = Synthetic Construct
  source 1..20: mol_type = other RNA
actcccacctaagggaatta

SEQ ID NO: 64 - RNA, 18 nt, synthetic construct
  misc_feature 1..18: note = Synthetic Construct
  source 1..18: mol_type = other RNA
ctcccacctaagggaatt

SEQ ID NO: 65 - RNA, 19 nt, synthetic construct
  misc_feature 1..19: note = Synthetic Construct
  source 1..19: mol_type = other RNA
ctcccacctaagggaatta

SEQ ID NO: 66 - RNA, 18 nt, synthetic construct
  misc_feature 1..18: note = Synthetic Construct
  source 1..18: mol_type = other RNA
tcccacctaagggaatta

SEQ ID NO: 67 - DNA, 18 bp, synthetic construct
  misc_feature 1..18: note = Synthetic Construct
  source 1..18: mol_type = other DNA
acatctcttggcagcatg

SEQ ID NO: 68 - DNA, 19 bp, synthetic construct
  misc_feature 1..19: note = Synthetic Construct
  source 1..19: mol_type = other DNA
cacatctcttggcagcatg

SEQ ID NO: 69 - DNA, 20 bp, synthetic construct
  misc_feature 1..20: note = Synthetic Construct
  source 1..20: mol_type = other DNA
gcacatctcttggcagcatg

SEQ ID NO: 70 - DNA, 18 bp, synthetic construct
  misc_feature 1..18: note = Synthetic Construct
  source 1..18: mol_type = other DNA
cacatctcttggcagcat

SEQ ID NO: 71 - DNA, 19 bp, synthetic construct
  misc_feature 1..19: note = Synthetic Construct
  source 1..19: mol_type = other DNA
gcacatctcttggcagcat

SEQ ID NO: 72 - DNA, 20 bp, synthetic construct
  misc_feature 1..20: note = Synthetic Construct
  source 1..20: mol_type = other DNA
ggcacatctcttggcagcat

SEQ ID NO: 73 - DNA, 19 bp, synthetic construct
  misc_feature 1..19: note = Synthetic Construct
  source 1..19: mol_type = other DNA
ggcacatctcttggcagca

SEQ ID NO: 74 - DNA, 20 bp, synthetic construct
  misc_feature 1..20: note = Synthetic Construct
  source 1..20: mol_type = other DNA
tggcacatctcttggcagca

SEQ ID NO: 75 - DNA, 19 bp, synthetic construct
  misc_feature 1..19: note = Synthetic Construct
  source 1..19: mol_type = other DNA
tggcacatctcttggcagc

SEQ ID NO: 76 - DNA, 20 bp, synthetic construct
  misc_feature 1..20: note = Synthetic Construct
  source 1..20: mol_type = other DNA
atggcacatctcttggcagc

SEQ ID NO: 77 - DNA, 18 bp, synthetic construct
  misc_feature 1..18: note = Synthetic Construct
  source 1..18: mol_type = other DNA
tggcacatctcttggcag

SEQ ID NO: 78 - DNA, 19 bp, synthetic construct
  misc_feature 1..19: note = Synthetic Construct
  source 1..19: mol_type = other DNA
atggcacatctcttggcag

SEQ ID NO: 79 - DNA, 20 bp, synthetic construct
  misc_feature 1..20: note = Synthetic Construct
  source 1..20: mol_type = other DNA
aatggcacatctcttggcag

SEQ ID NO: 80 - DNA, 18 bp, synthetic construct
  misc_feature 1..18: note = Synthetic Construct
  source 1..18: mol_type = other DNA
atggcacatctcttggca

SEQ ID NO: 81 - DNA, 19 bp, synthetic construct
  misc_feature 1..19: note = Synthetic Construct
  source 1..19: mol_type = other DNA
aatggcacatctcttggca

SEQ ID NO: 82 - DNA, 20 bp, synthetic construct
  misc_feature 1..20: note = Synthetic Construct
  source 1..20: mol_type = other DNA
gaatggcacatctcttggca

SEQ ID NO: 83 - DNA, 18 bp, synthetic construct
  misc_feature 1..18: note = Synthetic Construct
  source 1..18: mol_type = other DNA
aatggcacatctcttggc

SEQ ID NO: 84 - DNA, 19 bp, synthetic construct
  misc_feature 1..19: note = Synthetic Construct
  source 1..19: mol_type = other DNA
gaatggcacatctcttggc

SEQ ID NO: 85 - DNA, 20 bp, synthetic construct
  misc_feature 1..20: note = Synthetic Construct
  source 1..20: mol_type = other DNA
agaatggcacatctcttggc

SEQ ID NO: 86 - DNA, 18 bp, synthetic construct
  misc_feature 1..18: note = Synthetic Construct
  source 1..18: mol_type = other DNA
gaatggcacatctcttgg

SEQ ID NO: 87 - DNA, 19 bp, synthetic construct
  misc_feature 1..19: note = Synthetic Construct
  source 1..19: mol_type = other DNA
agaatggcacatctcttgg

SEQ ID NO: 88 - DNA, 20 bp, synthetic construct
  misc_feature 1..20: note = Synthetic Construct
  source 1..20: mol_type = other DNA
tagaatggcacatctcttgg

SEQ ID NO: 89 - DNA, 18 bp, synthetic construct
  misc_feature 1..18: note = Synthetic Construct
  source 1..18: mol_type = other DNA
agaatggcacatctcttg

SEQ ID NO: 90 - DNA, 19 bp, synthetic construct
  misc_feature 1..19: note = Synthetic Construct
  source 1..19: mol_type = other DNA
tagaatggcacatctcttg

SEQ ID NO: 91 - DNA, 20 bp, synthetic construct
  misc_feature 1..20: note = Synthetic Construct
  source 1..20: mol_type = other DNA
atagaatggcacatctcttg

SEQ ID NO: 92 - DNA, 18 bp, synthetic construct
  misc_feature 1..18: note = Synthetic Construct
  source 1..18: mol_type = other DNA
atacacgtcggtaaagga

SEQ ID NO: 93 - DNA, 19 bp, synthetic construct
  misc_feature 1..19: note = Synthetic Construct
  source 1..19: mol_type = other DNA
tatacacgtcggtaaagga

SEQ ID NO: 94 - DNA, 20 bp, synthetic construct
  misc_feature 1..20: note = Synthetic Construct
  source 1..20: mol_type = other DNA
atatacacgtcggtaaagga

SEQ ID NO: 95 - DNA, 18 bp, synthetic construct
  misc_feature 1..18: note = Synthetic Construct
  source 1..18: mol_type = other DNA
tatacacgtcggtaaagg

SEQ ID NO: 96 - DNA, 19 bp, synthetic construct
  misc_feature 1..19: note = Synthetic Construct
  source 1..19: mol_type = other DNA
atatacacgtcggtaaagg

SEQ ID NO: 97 - DNA, 20 bp, synthetic construct
  misc_feature 1..20: note = Synthetic Construct
  source 1..20: mol_type = other DNA
aatatacacgtcggtaaagg

SEQ ID NO: 98 - DNA, 20 bp, synthetic construct
  misc_feature 1..20: note = Synthetic Construct
  source 1..20: mol_type = other DNA
gatagaatatacacgtcggt

SEQ ID NO: 99 - DNA, 19 bp, synthetic construct
  misc_feature 1..19: note = Synthetic Construct
  source 1..19: mol_type = other DNA
gatagaatatacacgtcgg

SEQ ID NO: 100 - DNA, 20 bp, synthetic construct
  misc_feature 1..20: note = Synthetic Construct
  source 1..20: mol_type = other DNA
agatagaatatacacgtcgg

SEQ ID NO: 101 - DNA, 20 bp, synthetic construct
  misc_feature 1..20: note = Synthetic Construct
  source 1..20: mol_type = other DNA
ccatagctcaatgttctaga

SEQ ID NO: 102 - DNA, 18 bp, synthetic construct
  misc_feature 1..18: note = Synthetic Construct
  source 1..18: mol_type = other DNA
gtcttccatagctcaatg

SEQ ID NO: 103 - DNA, 20 bp, synthetic construct
  misc_feature 1..20: note = Synthetic Construct
  source 1..20: mol_type = other DNA
taggtgggagtcttccatag

SEQ ID NO: 104 - DNA, 19 bp, synthetic construct
  misc_feature 1..19: note = Synthetic Construct
  source 1..19: mol_type = other DNA
taggtgggagtcttccata

SEQ ID NO: 105 - DNA, 20 bp, synthetic construct
  misc_feature 1..20: note = Synthetic Construct
  source 1..20: mol_type = other DNA
ttaggtgggagtcttccata

SEQ ID NO: 106 - DNA, 18 bp, synthetic construct
  misc_feature 1..18: note = Synthetic Construct
  source 1..18: mol_type = other DNA
taggtgggagtcttccat

SEQ ID NO: 107 - DNA, 19 bp, synthetic construct
  misc_feature 1..19: note = Synthetic Construct
  source 1..19: mol_type = other DNA
ttaggtgggagtcttccat

SEQ ID NO: 108 - DNA, 18 bp, synthetic construct
  misc_feature 1..18: note = Synthetic Construct
  source 1..18: mol_type = other DNA
ttaggtgggagtcttcca

SEQ ID NO: 109 - DNA, 20 bp, synthetic construct
  misc_feature 1..20: note = Synthetic Construct
  source 1..20: mol_type = other DNA
aattcccttaggtgggagtc

SEQ ID NO: 110 - DNA, 18 bp, synthetic construct
  misc_feature 1..18: note = Synthetic Construct
  source 1..18: mol_type = other DNA
attcccttaggtgggagt

SEQ ID NO: 111 - DNA, 19 bp, synthetic construct
  misc_feature 1..19: note = Synthetic Construct
  source 1..19: mol_type = other DNA
aattcccttaggtgggagt

SEQ ID NO: 112 - DNA, 20 bp, synthetic construct
  misc_feature 1..20: note = Synthetic Construct
  source 1..20: mol_type = other DNA
taattcccttaggtgggagt

SEQ ID NO: 113 - DNA, 18 bp, synthetic construct
  misc_feature 1..18: note = Synthetic Construct
  source 1..18: mol_type = other DNA
aattcccttaggtgggag

SEQ ID NO: 114 - DNA, 19 bp, synthetic construct
  misc_feature 1..19: note = Synthetic Construct
  source 1..19: mol_type = other DNA
taattcccttaggtgggag

SEQ ID NO: 115 - DNA, 18 bp, synthetic construct
  misc_feature 1..18: note = Synthetic Construct
  source 1..18: mol_type = other DNA
taattcccttaggtggga

SEQ ID NO: 116 - RNA, 20 nt, synthetic construct
  misc_feature 1..20: note = Synthetic Construct
  source 1..20: mol_type = other RNA
gataaagactgctgagaaga

SEQ ID NO: 117 - RNA, 20 nt, synthetic construct
  misc_feature 1..20: note = Synthetic Construct
  source 1..20: mol_type = other RNA
ataaagactgctgagaagag

SEQ ID NO: 118 - RNA, 20 nt, synthetic construct
  misc_feature 1..20: note = Synthetic Construct
  source 1..20: mol_type = other RNA
taaagactgctgagaagagc

SEQ ID NO: 119 - RNA, 20 nt, synthetic construct
  misc_feature 1..20: note = Synthetic Construct
  source 1..20: mol_type = other RNA
aaagactgctgagaagagca

SEQ ID NO: 120 - RNA, 20 nt, synthetic construct
  misc_feature 1..20: note = Synthetic Construct
  source 1..20: mol_type = other RNA
aagactgctgagaagagcac

SEQ ID NO: 121 - RNA, 20 nt, synthetic construct
  misc_feature 1..20: note = Synthetic Construct
  source 1..20: mol_type = other RNA
agactgctgagaagagcacc

SEQ ID NO: 122 - RNA, 20 nt, synthetic construct
  misc_feature 1..20: note = Synthetic Construct
  source 1..20: mol_type = other RNA
gactgctgagaagagcaccc

SEQ ID NO: 123 - RNA, 20 nt, synthetic construct
  misc_feature 1..20: note = Synthetic Construct
  source 1..20: mol_type = other RNA
caagtgctaccgcacaggca

SEQ ID NO: 124 - RNA, 20 nt, synthetic construct
  misc_feature 1..20: note = Synthetic Construct
  source 1..20: mol_type = other RNA
aagtgctaccgcacaggcat

SEQ ID NO: 125 - RNA, 20 nt, synthetic construct
  misc_feature 1..20: note = Synthetic Construct
  source 1..20: mol_type = other RNA
agtgctaccgcacaggcatg

SEQ ID NO: 126 - RNA, 20 nt, synthetic construct
  misc_feature 1..20: note = Synthetic Construct
  source 1..20: mol_type = other RNA
tgctaccgcacaggcatgct

SEQ ID NO: 127 - RNA, 20 nt, synthetic construct
  misc_feature 1..20: note = Synthetic Construct
  source 1..20: mol_type = other RNA
taccgcacaggcatgctgca

SEQ ID NO: 128 - RNA, 20 nt, synthetic construct
  misc_feature 1..20: note = Synthetic Construct
  source 1..20: mol_type = other RNA
gcacaggcatgctgcagtga

SEQ ID NO: 129 - RNA, 20 nt, synthetic construct
  misc_feature 1..20: note = Synthetic Construct
  source 1..20: mol_type = other RNA
cacaggcatgctgcagtgaa

SEQ ID NO: 130 - RNA, 20 nt, synthetic construct
  misc_feature 1..20: note = Synthetic Construct
  source 1..20: mol_type = other RNA
acaggcatgctgcagtgaat

SEQ ID NO: 131 - RNA, 20 nt, synthetic construct
  misc_feature 1..20: note = Synthetic Construct
  source 1..20: mol_type = other RNA
caggcatgctgcagtgaatt

SEQ ID NO: 132 - RNA, 20 nt, synthetic construct
  misc_feature 1..20: note = Synthetic Construct
  source 1..20: mol_type = other RNA
aggcatgctgcagtgaattt

SEQ ID NO: 133 - RNA, 20 nt, synthetic construct
  misc_feature 1..20: note = Synthetic Construct
  source 1..20: mol_type = other RNA
ggcatgctgcagtgaattta

SEQ ID NO: 134 - RNA, 20 nt, synthetic construct
  misc_feature 1..20: note = Synthetic Construct
  source 1..20: mol_type = other RNA
gcatgctgcagtgaatttaa

SEQ ID NO: 135 - RNA, 20 nt, synthetic construct
  misc_feature 1..20: note = Synthetic Construct
  source 1..20: mol_type = other RNA
catgctgcagtgaatttaac

SEQ ID NO: 136 - RNA, 20 nt, synthetic construct
  misc_feature 1..20: note = Synthetic Construct
  source 1..20: mol_type = other RNA
gcagtgaatttaactgatcc

SEQ ID NO: 137 - RNA, 20 nt, synthetic construct
  misc_feature 1..20: note = Synthetic Construct
  source 1..20: mol_type = other RNA
tccctgcaaccgttgtttaa

SEQ ID NO: 138 - RNA, 20 nt, synthetic construct
  misc_feature 1..20: note = Synthetic Construct
  source 1..20: mol_type = other RNA
ccctgcaaccgttgtttaag

SEQ ID NO: 139 - DNA, 20 bp, synthetic construct
  misc_feature 1..20: note = Synthetic Construct
  source 1..20: mol_type = other DNA
tcttctcagcagtctttatc

SEQ ID NO: 140 - DNA, 20 bp, synthetic construct
  misc_feature 1..20: note = Synthetic Construct
  source 1..20: mol_type = other DNA
ctcttctcagcagtctttat

SEQ ID NO: 141 - DNA, 20 bp, synthetic construct
  misc_feature 1..20: note = Synthetic Construct
  source 1..20: mol_type = other DNA
gctcttctcagcagtcttta

SEQ ID NO: 142 - DNA, 20 bp, synthetic construct
  misc_feature 1..20: note = Synthetic Construct
  source 1..20: mol_type = other DNA
tgctcttctcagcagtcttt

SEQ ID NO: 143 - DNA, 20 bp, synthetic construct
  misc_feature 1..20: note = Synthetic Construct
  source 1..20: mol_type = other DNA
gtgctcttctcagcagtctt

SEQ ID NO: 144 - DNA, 20 bp, synthetic construct
  misc_feature 1..20: note = Synthetic Construct
  source 1..20: mol_type = other DNA
ggtgctcttctcagcagtct

SEQ ID NO: 145 - DNA, 20 bp, synthetic construct
  misc_feature 1..20: note = Synthetic Construct
  source 1..20: mol_type = other DNA
gggtgctcttctcagcagtc

SEQ ID NO: 146 - DNA, 20 bp, synthetic construct
  misc_feature 1..20: note = Synthetic Construct
  source 1..20: mol_type = other DNA
tgcctgtgcggtagcacttg

SEQ ID NO: 147 - DNA, 20 bp, synthetic construct
  misc_feature 1..20: note = Synthetic Construct
  source 1..20: mol_type = other DNA
atgcctgtgcggtagcactt

SEQ ID NO: 148 - DNA, 20 bp, synthetic construct
  misc_feature 1..20: note = Synthetic Construct
  source 1..20: mol_type = other DNA
catgcctgtgcggtagcact

SEQ ID NO: 149 - DNA, 20 bp, synthetic construct
  misc_feature 1..20: note = Synthetic Construct
  source 1..20: mol_type = other DNA
agcatgcctgtgcggtagca

SEQ ID NO: 150 - DNA, 20 bp, synthetic construct
  misc_feature 1..20: note = Synthetic Construct
  source 1..20: mol_type = other DNA
tgcagcatgcctgtgcggta

SEQ ID NO: 151 - DNA, 20 bp, synthetic construct
  misc_feature 1..20: note = Synthetic Construct
  source 1..20: mol_type = other DNA
tcactgcagcatgcctgtgc

SEQ ID NO: 152 - DNA, 20 bp, synthetic construct
  misc_feature 1..20: note = Synthetic Construct
  source 1..20: mol_type = other DNA
ttcactgcagcatgcctgtg

SEQ ID NO: 153 - DNA, 20 bp, synthetic construct
  misc_feature 1..20: note = Synthetic Construct
  source 1..20: mol_type = other DNA
attcactgcagcatgcctgt

SEQ ID NO: 154 - DNA, 20 bp, synthetic construct
  misc_feature 1..20: note = Synthetic Construct
  source 1..20: mol_type = other DNA
aattcactgcagcatgcctg

SEQ ID NO: 155 - DNA, 20 bp, synthetic construct
  misc_feature 1..20: note = Synthetic Construct
  source 1..20: mol_type = other DNA
aaattcactgcagcatgcct

SEQ ID NO: 156 - DNA, 20 bp, synthetic construct
  misc_feature 1..20: note = Synthetic Construct
  source 1..20: mol_type = other DNA
taaattcactgcagcatgcc

SEQ ID NO: 157 - DNA, 20 bp, synthetic construct
  misc_feature 1..20: note = Synthetic Construct
  source 1..20: mol_type = other DNA
ttaaattcactgcagcatgc

SEQ ID NO: 158 - DNA, 20 bp, synthetic construct
  misc_feature 1..20: note = Synthetic Construct
  source 1..20: mol_type = other DNA
gttaaattcactgcagcatg

SEQ ID NO: 159 - DNA, 20 bp, synthetic construct
  misc_feature 1..20: note = Synthetic Construct
  source 1..20: mol_type = other DNA
ggatcagttaaattcactgc

SEQ ID NO: 160 - DNA, 20 bp, synthetic construct
  misc_feature 1..20: note = Synthetic Construct
  source 1..20: mol_type = other DNA
ttaaacaacggttgcaggga

SEQ ID NO: 161 - DNA, 20 bp, synthetic construct
  misc_feature 1..20: note = Synthetic Construct
  source 1..20: mol_type = other DNA
cttaaacaacggttgcaggg

SEQ ID NO: 162 - RNA, 19 nt, synthetic construct
  misc_feature 1..19: note = Synthetic Construct
  source 1..19: mol_type = other RNA
aaaagactgtggaggaaga

SEQ ID NO: 163 - RNA, 20 nt, synthetic construct
  misc_feature 1..20: note = Synthetic Construct
  source 1..20: mol_type = other RNA
aaaagactgtggaggaagaa

SEQ ID NO: 164 - RNA, 19 nt, synthetic construct
  misc_feature 1..19: note = Synthetic Construct
  source 1..19: mol_type = other RNA
aaagactgtggaggaagaa

SEQ ID NO: 165 - RNA, 20 nt, synthetic construct
  misc_feature 1..20: note = Synthetic Construct
  source 1..20: mol_type = other RNA
aaagactgtggaggaagaaa

SEQ ID NO: 166 - RNA, 20 nt, synthetic construct
  misc_feature 1..20: note = Synthetic Construct
  source 1..20: mol_type = other RNA
aagactgtggaggaagaaaa

SEQ ID NO: 167 - RNA, 20 nt, synthetic construct
  misc_feature 1..20: note = Synthetic Construct
  source 1..20: mol_type = other RNA
agactgtggaggaagaaaac

SEQ ID NO: 168 - RNA, 18 nt, synthetic construct
  misc_feature 1..18: note = Synthetic Construct
  source 1..18: mol_type = other RNA
actgtggaggaagaaaac

SEQ ID NO: 169 - RNA, 19 nt, synthetic construct
  misc_feature 1..19: note = Synthetic Construct
  source 1..19: mol_type = other RNA
actgtggaggaagaaaacc

SEQ ID NO: 170 - RNA, 20 nt, synthetic construct
  misc_feature 1..20: note = Synthetic Construct
  source 1..20: mol_type = other RNA
actgtggaggaagaaaaccc

SEQ ID NO: 171 - RNA, 18 nt, synthetic construct
  misc_feature 1..18: note = Synthetic Construct
  source 1..18: mol_type = other RNA
ctgtggaggaagaaaacc

SEQ ID NO: 172 - RNA, 19 nt, synthetic construct
  misc_feature 1..19: note = Synthetic Construct
  source 1..19: mol_type = other RNA
ctgtggaggaagaaaaccc

SEQ ID NO: 173 - RNA, 19 nt, synthetic construct
  misc_feature 1..19: note = Synthetic Construct
  source 1..19: mol_type = other RNA
aaaaccctttaccctgttg

SEQ ID NO: 174 - RNA, 20 nt, synthetic construct
  misc_feature 1..20: note = Synthetic Construct
  source 1..20: mol_type = other RNA
aaaaccctttaccctgttgt

SEQ ID NO: 175 - RNA, 20 nt, synthetic construct
  misc_feature 1..20: note = Synthetic Construct
  source 1..20: mol_type = other RNA
aaaccctttaccctgttgtt

SEQ ID NO: 176 - RNA, 18 nt, synthetic construct
  misc_feature 1..18: note = Synthetic Construct
  source 1..18: mol_type = other RNA
ttgttcagggagaaactg

SEQ ID NO: 177 - RNA, 20 nt, synthetic construct
  misc_feature 1..20: note = Synthetic Construct
  source 1..20: mol_type = other RNA
ttgttcagggagaaactgac

SEQ ID NO: 178 - RNA, 18 nt, synthetic construct
  misc_feature 1..18: note = Synthetic Construct
  source 1..18: mol_type = other RNA
tgttcagggagaaactga

SEQ ID NO: 179 - RNA, 19 nt, synthetic construct
  misc_feature 1..19: note = Synthetic Construct
  source 1..19: mol_type = other RNA
tgttcagggagaaactgac

SEQ ID NO: 180 - RNA, 20 nt, synthetic construct
  misc_feature 1..20: note = Synthetic Construct
  source 1..20: mol_type = other RNA
tgttcagggagaaactgaca

SEQ ID NO: 181 - RNA, 19 nt, synthetic construct
  misc_feature 1..19: note = Synthetic Construct
  source 1..19: mol_type = other RNA
gttcagggagaaactgaca

SEQ ID NO: 182 - RNA, 20 nt, synthetic construct
  misc_feature 1..20: note = Synthetic Construct
  source 1..20: mol_type = other RNA
tcagggagaaactgacacca

SEQ ID NO: 183 - RNA, 19 nt, synthetic construct
  misc_feature 1..19: note = Synthetic Construct
  source 1..19: mol_type = other RNA
cagggagaaactgacacca

SEQ ID NO: 184 - RNA, 18 nt, synthetic construct
  misc_feature 1..18: note = Synthetic Construct
  source 1..18: mol_type = other RNA
agggagaaactgacacca

SEQ ID NO: 185 - RNA, 19 nt, synthetic construct
  misc_feature 1..19: note = Synthetic Construct
  source 1..19: mol_type = other RNA
agggagaaactgacaccac

SEQ ID NO: 186 - RNA, 20 nt, synthetic construct
  misc_feature 1..20: note = Synthetic Construct
  source 1..20: mol_type = other RNA
agggagaaactgacaccact

SEQ ID NO: 187 - RNA, 18 nt, synthetic construct
  misc_feature 1..18: note = Synthetic Construct
  source 1..18: mol_type = other RNA
gggagaaactgacaccac

SEQ ID NO: 188 - RNA, 19 nt, synthetic construct
  misc_feature 1..19: note = Synthetic Construct
  source 1..19: mol_type = other RNA
gggagaaactgacaccact

SEQ ID NO: 189 - RNA, 20 nt, synthetic construct
  misc_feature 1..20: note = Synthetic Construct
  source 1..20: mol_type = other RNA
gggagaaactgacaccactc

SEQ ID NO: 190 - RNA, 18 nt, synthetic construct
  misc_feature 1..18: note = Synthetic Construct
  source 1..18: mol_type = other RNA
ggagaaactgacaccact

SEQ ID NO: 191 - RNA, 19 nt, synthetic construct
  misc_feature 1..19: note = Synthetic Construct
  source 1..19: mol_type = other RNA
ggagaaactgacaccactc

SEQ ID NO: 192 - RNA, 20 nt, synthetic construct
  misc_feature 1..20: note = Synthetic Construct
  source 1..20: mol_type = other RNA
ggagaaactgacaccactca

SEQ ID NO: 193 - RNA, 18 nt, synthetic construct
  misc_feature 1..18: note = Synthetic Construct
  source 1..18: mol_type = other RNA
gagaaactgacaccactc

SEQ ID NO: 194 - RNA, 19 nt, synthetic construct
  misc_feature 1..19: note = Synthetic Construct
  source 1..19: mol_type = other RNA
gagaaactgacaccactca

SEQ ID NO: 195 - RNA, 20 nt, synthetic construct
  misc_feature 1..20: note = Synthetic Construct
  source 1..20: mol_type = other RNA
gagaaactgacaccactcaa

SEQ ID NO: 196 - RNA, 18 nt, synthetic construct
  misc_feature 1..18: note = Synthetic Construct
  source 1..18: mol_type = other RNA
agaaactgacaccactca

SEQ ID NO: 197 - RNA, 19 nt, synthetic construct
  misc_feature 1..19: note = Synthetic Construct
  source 1..19: mol_type = other RNA
agaaactgacaccactcaa

SEQ ID NO: 198 - RNA, 20 nt, synthetic construct
  misc_feature 1..20: note = Synthetic Construct
  source 1..20: mol_type = other RNA
agaaactgacaccactcaac

SEQ ID NO: 199 - RNA, 18 nt, synthetic construct
  misc_feature 1..18: note = Synthetic Construct
  source 1..18: mol_type = other RNA
gaaactgacaccactcaa

SEQ ID NO: 200 - RNA, 19 nt, synthetic construct
  misc_feature 1..19: note = Synthetic Construct
  source 1..19: mol_type = other RNA
gaaactgacaccactcaac

SEQ ID NO: 201 - RNA, 20 nt, synthetic construct
  misc_feature 1..20: note = Synthetic Construct
  source 1..20: mol_type = other RNA
gaaactgacaccactcaact

SEQ ID NO: 202 - RNA, 18 nt, synthetic construct
  misc_feature 1..18: note = Synthetic Construct
  source 1..18: mol_type = other RNA
aaactgacaccactcaac

SEQ ID NO: 203 - RNA, 19 nt, synthetic construct
  misc_feature 1..19: note = Synthetic Construct
  source 1..19: mol_type = other RNA
aaactgacaccactcaact

SEQ ID NO: 204 - RNA, 20 nt, synthetic construct
  misc_feature 1..20: note = Synthetic Construct
  source 1..20: mol_type = other RNA
aaactgacaccactcaactg

SEQ ID NO: 205 - RNA, 18 nt, synthetic construct
  misc_feature 1..18: note = Synthetic Construct
  source 1..18: mol_type = other RNA
aactgacaccactcaact

SEQ ID NO: 206 - RNA, 19 nt, synthetic construct
  misc_feature 1..19: note = Synthetic Construct
  source 1..19: mol_type = other RNA
aactgacaccactcaactg

SEQ ID NO: 207 - RNA, 20 nt, synthetic construct
  misc_feature 1..20: note = Synthetic Construct
  source 1..20: mol_type = other RNA
aactgacaccactcaactgc

SEQ ID NO: 208 - RNA, 18 nt, synthetic construct
  misc_feature 1..18: note = Synthetic Construct
  source 1..18: mol_type = other RNA
actgacaccactcaactg

SEQ ID NO: 209 - RNA, 19 nt, synthetic construct
  misc_feature 1..19: note = Synthetic Construct
  source 1..19: mol_type = other RNA
actgacaccactcaactgc

SEQ ID NO: 210 - RNA, 20 nt, synthetic construct
  misc_feature 1..20: note = Synthetic Construct
  source 1..20: mol_type = other RNA
actgacaccactcaactgcc

SEQ ID NO: 211 - RNA, 18 nt, synthetic construct
  misc_feature 1..18: note = Synthetic Construct
  source 1..18: mol_type = other RNA
ctgacaccactcaactgc

SEQ ID NO: 212 - RNA, 19 nt, synthetic construct
  misc_feature 1..19: note = Synthetic Construct
  source 1..19: mol_type = other RNA
ctgacaccactcaactgcc

SEQ ID NO: 213 - RNA, 20 nt, synthetic construct
  misc_feature 1..20: note = Synthetic Construct
  source 1..20: mol_type = other RNA
ctgacaccactcaactgcct

SEQ ID NO: 214 - RNA, 18 nt, synthetic construct
  misc_feature 1..18: note = Synthetic Construct
  source 1..18: mol_type = other RNA
tgacaccactcaactgcc

SEQ ID NO: 215 - RNA, 19 nt, synthetic construct
  misc_feature 1..19: note = Synthetic Construct
  source 1..19: mol_type = other RNA
tgacaccactcaactgcct

SEQ ID NO: 216 - RNA, 20 nt, synthetic construct
  misc_feature 1..20: note = Synthetic Construct
  source 1..20: mol_type = other RNA
tgacaccactcaactgcctg

SEQ ID NO: 217 - RNA, 18 nt, synthetic construct
  misc_feature 1..18: note = Synthetic Construct
  source 1..18: mol_type = other RNA
gacaccactcaactgcct

SEQ ID NO: 218 - RNA, 19 nt, synthetic construct
  misc_feature 1..19: note = Synthetic Construct
  source 1..19: mol_type = other RNA
gacaccactcaactgcctg

SEQ ID NO: 219 - RNA, 20 nt, synthetic construct
  misc_feature 1..20: note = Synthetic Construct
  source 1..20: mol_type = other RNA
gacaccactcaactgcctgg

SEQ ID NO: 220 - RNA, 18 nt, synthetic construct
  misc_feature 1..18: note = Synthetic Construct
  source 1..18: mol_type = other RNA
acaccactcaactgcctg

SEQ ID NO: 221 - RNA, 19 nt, synthetic construct
  misc_feature 1..19: note = Synthetic Construct
  source 1..19: mol_type = other RNA
acaccactcaactgcctgg

SEQ ID NO: 222 - RNA, 20 nt, synthetic construct
  misc_feature 1..20: note = Synthetic Construct
  source 1..20: mol_type = other RNA
acaccactcaactgcctggc

SEQ ID NO: 223 - RNA, 20 nt, synthetic construct
  misc_feature 1..20: note = Synthetic Construct
  source 1..20: mol_type = other RNA
caccactcaactgcctggca

SEQ ID NO: 224 - RNA, 18 nt, synthetic construct
  misc_feature 1..18: note = Synthetic Construct
  source 1..18: mol_type = other RNA
gaaaatgtggcatccagt

SEQ ID NO: 225 - RNA, 18 nt, synthetic construct
  misc_feature 1..18: note = Synthetic Construct
  source 1..18: mol_type = other RNA
aaaatgtggcatccagtc

SEQ ID NO: 226 - RNA, 20 nt, synthetic construct
  misc_feature 1..20: note = Synthetic Construct
  source 1..20: mol_type = other RNA
gcatccagtccactttacca

SEQ ID NO: 227 - RNA, 18 nt, synthetic construct
  misc_feature 1..18: note = Synthetic Construct
  source 1..18: mol_type = other RNA
catccagtccactttacc

SEQ ID NO: 228 - RNA, 19 nt, synthetic construct
  misc_feature 1..19: note = Synthetic Construct
  source 1..19: mol_type = other RNA
catccagtccactttacca

SEQ ID NO: 229 - RNA, 20 nt, synthetic construct
  misc_feature 1..20: note = Synthetic Construct
  source 1..20: mol_type = other RNA
catccagtccactttaccat

SEQ ID NO: 230 - RNA, 18 nt, synthetic construct
  misc_feature 1..18: note = Synthetic Construct
  source 1..18: mol_type = other RNA
atccagtccactttacca

SEQ ID NO: 231 - RNA, 19 nt, synthetic construct
  misc_feature 1..19: note = Synthetic Construct
  source 1..19: mol_type = other RNA
atccagtccactttaccat

SEQ ID NO: 232 - RNA, 20 nt, synthetic construct
  misc_feature 1..20: note = Synthetic Construct
  source 1..20: mol_type = other RNA
atccagtccactttaccatc

SEQ ID NO: 233 - RNA, 20 nt, synthetic construct
  misc_feature 1..20: note = Synthetic Construct
  source 1..20: mol_type = other RNA
gtttaaggaaaccatctctg

SEQ ID NO: 234 - RNA, 20 nt, synthetic construct
  misc_feature 1..20: note = Synthetic Construct
  source 1..20: mol_type = other RNA
tttaaggaaaccatctctgg

SEQ ID NO: 235 - RNA, 19 nt, synthetic construct
  misc_feature 1..19: note = Synthetic Construct
  source 1..19: mol_type = other RNA
ttaaggaaaccatctctgg

SEQ ID NO: 236 - RNA, 18 nt, synthetic construct
  misc_feature 1..18: note = Synthetic Construct
  source 1..18: mol_type = other RNA
taaggaaaccatctctgg

SEQ ID NO: 237 - DNA, 19 bp, synthetic construct
  misc_feature 1..19: note = Synthetic Construct
  source 1..19: mol_type = other DNA
tcttcctccacagtctttt

SEQ ID NO: 238 - DNA, 20 bp, synthetic construct
  misc_feature 1..20: note = Synthetic Construct
  source 1..20: mol_type = other DNA
ttcttcctccacagtctttt

SEQ ID NO: 239 - DNA, 19 bp, synthetic construct
  misc_feature 1..19: note = Synthetic Construct
  source 1..19: mol_type = other DNA
ttcttcctccacagtcttt

SEQ ID NO: 240 - DNA, 20 bp, synthetic construct
  misc_feature 1..20: note = Synthetic Construct
  source 1..20: mol_type = other DNA
tttcttcctccacagtcttt

SEQ ID NO: 241 - DNA, 20 bp, synthetic construct
  misc_feature 1..20: note = Synthetic Construct
  source 1..20: mol_type = other DNA
ttttcttcctccacagtctt

SEQ ID NO: 242 - DNA, 20 bp, synthetic construct
  misc_feature 1..20: note = Synthetic Construct
  source 1..20: mol_type = other DNA
gttttcttcctccacagtct

SEQ ID NO: 243 - DNA, 18 bp, synthetic construct
  misc_feature 1..18: note = Synthetic Construct
  source 1..18: mol_type = other DNA
gttttcttcctccacagt

SEQ ID NO: 244 - DNA, 19 bp, synthetic construct
  misc_feature 1..19: note = Synthetic Construct
  source 1..19: mol_type = other DNA
ggttttcttcctccacagt

SEQ ID NO: 245 - DNA, 20 bp, synthetic construct
  misc_feature 1..20: note = Synthetic Construct
  source 1..20: mol_type = other DNA
gggttttcttcctccacagt

SEQ ID NO: 246 - DNA, 18 bp, synthetic construct
  misc_feature 1..18: note = Synthetic Construct
  source 1..18: mol_type = other DNA
ggttttcttcctccacag

SEQ ID NO: 247 - DNA, 19 bp, synthetic construct
  misc_feature 1..19: note = Synthetic Construct
  source 1..19: mol_type = other DNA
gggttttcttcctccacag

SEQ ID NO: 248 - DNA, 19 bp, synthetic construct
  misc_feature 1..19: note = Synthetic Construct
  source 1..19: mol_type = other DNA
caacagggtaaagggtttt

SEQ ID NO: 249 - DNA, 20 bp, synthetic construct
  misc_feature 1..20: note = Synthetic Construct
  source 1..20: mol_type = other DNA
acaacagggtaaagggtttt

SEQ ID NO: 250 - DNA, 20 bp, synthetic construct
  misc_feature 1..20: note = Synthetic Construct
  source 1..20: mol_type = other DNA
aacaacagggtaaagggttt

SEQ ID NO: 251 - DNA, 18 bp, synthetic construct
  misc_feature 1..18: note = Synthetic Construct
  source 1..18: mol_type = other DNA
cagtttctccctgaacaa

SEQ ID NO: 252 - DNA, 20 bp, synthetic construct
  misc_feature 1..20: note = Synthetic Construct
  source 1..20: mol_type = other DNA
gtcagtttctccctgaacaa

SEQ ID NO: 253 - DNA, 18 bp, synthetic construct
  misc_feature 1..18: note = Synthetic Construct
  source 1..18: mol_type = other DNA
tcagtttctccctgaaca

SEQ ID NO: 254 - DNA, 19 bp, synthetic construct
  misc_feature 1..19: note = Synthetic Construct
  source 1..19: mol_type = other DNA
gtcagtttctccctgaaca

SEQ ID NO: 255 - DNA, 20 bp, synthetic construct
  misc_feature 1..20: note = Synthetic Construct
  source 1..20: mol_type = other DNA
tgtcagtttctccctgaaca

SEQ ID NO: 256 - DNA, 19 bp, synthetic construct
  misc_feature 1..19: note = Synthetic Construct
  source 1..19: mol_type = other DNA
tgtcagtttctccctgaac

SEQ ID NO: 257 - DNA, 20 bp, synthetic construct
  misc_feature 1..20: note = Synthetic Construct
  source 1..20: mol_type = other DNA
tggtgtcagtttctccctga

SEQ ID NO: 258 - DNA, 19 bp, synthetic construct
  misc_feature 1..19: note = Synthetic Construct
  source 1..19: mol_type = other DNA
tggtgtcagtttctccctg

SEQ ID NO: 259 - DNA, 18 bp, synthetic construct
  misc_feature 1..18: note = Synthetic Construct
  source 1..18: mol_type = other DNA
tggtgtcagtttctccct

SEQ ID NO: 260 - DNA, 19 bp, synthetic construct
  misc_feature 1..19: note = Synthetic Construct
  source 1..19: mol_type = other DNA
gtggtgtcagtttctccct

SEQ ID NO: 261 - DNA, 20 bp, synthetic construct
  misc_feature 1..20: note = Synthetic Construct
  source 1..20: mol_type = other DNA
agtggtgtcagtttctccct

SEQ ID NO: 262 - DNA, 18 bp, synthetic construct
  misc_feature 1..18: note = Synthetic Construct
  source 1..18: mol_type = other DNA
gtggtgtcagtttctccc

SEQ ID NO: 263 - DNA, 19 bp, synthetic construct
  misc_feature 1..19: note = Synthetic Construct
  source 1..19: mol_type = other DNA
agtggtgtcagtttctccc

SEQ ID NO: 264 - DNA, 20 bp, synthetic construct
  misc_feature 1..20: note = Synthetic Construct
  source 1..20: mol_type = other DNA
gagtggtgtcagtttctccc

SEQ ID NO: 265 - DNA, 18 bp, synthetic construct
  misc_feature 1..18: note = Synthetic Construct
  source 1..18: mol_type = other DNA
agtggtgtcagtttctcc

SEQ ID NO: 266 - DNA, 19 bp, synthetic construct
  misc_feature 1..19: note = Synthetic Construct
  source 1..19: mol_type = other DNA
gagtggtgtcagtttctcc

SEQ ID NO: 267 - DNA, 20 bp, synthetic construct
  misc_feature 1..20: note = Synthetic Construct
  source 1..20: mol_type = other DNA
tgagtggtgtcagtttctcc

SEQ ID NO: 268 - DNA, 18 bp, synthetic construct
  misc_feature 1..18: note = Synthetic Construct
  source 1..18: mol_type = other DNA
gagtggtgtcagtttctc

SEQ ID NO: 269 - DNA, 19 bp, synthetic construct
  misc_feature 1..19: note = Synthetic Construct
  source 1..19: mol_type = other DNA
tgagtggtgtcagtttctc

SEQ ID NO: 270 - DNA, 20 bp, synthetic construct
  misc_feature 1..20: note = Synthetic Construct
  source 1..20: mol_type = other DNA
ttgagtggtgtcagtttctc

SEQ ID NO: 271 - DNA, 18 bp, synthetic construct
  misc_feature 1..18: note = Synthetic Construct
  source 1..18: mol_type = other DNA
tgagtggtgtcagtttct

SEQ ID NO: 272 - DNA, 19 bp, synthetic construct
  misc_feature 1..19: note = Synthetic Construct
  source 1..19: mol_type = other DNA
ttgagtggtgtcagtttct

SEQ ID NO: 273 - DNA, 20 bp, synthetic construct
  misc_feature 1..20: note = Synthetic Construct
  source 1..20: mol_type = other DNA
gttgagtggtgtcagtttct

SEQ ID NO: 274 - DNA, 18 bp, synthetic construct
  misc_feature 1..18: note = Synthetic Construct
  source 1..18: mol_type = other DNA
ttgagtggtgtcagtttc

SEQ ID NO: 275 - DNA, 19 bp, synthetic construct
  misc_feature 1..19: note = Synthetic Construct
  source 1..19: mol_type = other DNA
gttgagtggtgtcagtttc

SEQ ID NO: 276 - DNA, 20 bp, synthetic construct
  misc_feature 1..20: note = Synthetic Construct
  source 1..20: mol_type = other DNA
agttgagtggtgtcagtttc

SEQ ID NO: 277 - DNA, 18 bp, synthetic construct
  misc_feature 1..18: note = Synthetic Construct
  source 1..18: mol_type = other DNA
gttgagtggtgtcagttt

SEQ ID NO: 278 - DNA, 19 bp, synthetic construct
  misc_feature 1..19: note = Synthetic Construct
  source 1..19: mol_type = other DNA
agttgagtggtgtcagttt

SEQ ID NO: 279 - DNA, 20 bp, synthetic construct
  misc_feature 1..20: note = Synthetic Construct
  source 1..20: mol_type = other DNA
cagttgagtggtgtcagttt

SEQ ID NO: 280 - DNA, 18 bp, synthetic construct
  misc_feature 1..18: note = Synthetic Construct
  source 1..18: mol_type = other DNA
agttgagtggtgtcagtt

SEQ ID NO: 281 - DNA, 19 bp, synthetic construct
  misc_feature 1..19: note = Synthetic Construct
  source 1..19: mol_type = other DNA
cagttgagtggtgtcagtt

SEQ ID NO: 282 - DNA, 20 bp, synthetic construct
  misc_feature 1..20: note = Synthetic Construct
  source 1..20: mol_type = other DNA
gcagttgagtggtgtcagtt

SEQ ID NO: 283 - DNA, 18 bp, synthetic construct
  misc_feature 1..18: note = Synthetic Construct
  source 1..18: mol_type = other DNA
cagttgagtggtgtcagt

SEQ ID NO: 284 - DNA, 19 bp, synthetic construct
  misc_feature 1..19: note = Synthetic Construct
  source 1..19: mol_type = other DNA
gcagttgagtggtgtcagt

SEQ ID NO: 285 - DNA, 20 bp, synthetic construct
  misc_feature 1..20: note = Synthetic Construct
  source 1..20: mol_type = other DNA
ggcagttgagtggtgtcagt

SEQ ID NO: 286 - DNA, 18 bp, synthetic construct
  misc_feature 1..18: note = Synthetic Construct
  source 1..18: mol_type = other DNA
gcagttgagtggtgtcag

SEQ ID NO: 287 - DNA, 19 bp, synthetic construct
  misc_feature 1..19: note = Synthetic Construct
  source 1..19: mol_type = other DNA
ggcagttgagtggtgtcag

SEQ ID NO: 288 - DNA, 20 bp, synthetic construct
  misc_feature 1..20: note = Synthetic Construct
  source 1..20: mol_type = other DNA
aggcagttgagtggtgtcag

SEQ ID NO: 289 - DNA, 18 bp, synthetic construct
  misc_feature 1..18: note = Synthetic Construct
  source 1..18: mol_type = other DNA
ggcagttgagtggtgtca

SEQ ID NO: 290 - DNA, 19 bp, synthetic construct
  misc_feature 1..19: note = Synthetic Construct
  source 1..19: mol_type = other DNA
aggcagttgagtggtgtca

SEQ ID NO: 291 - DNA, 20 bp, synthetic construct
  misc_feature 1..20: note = Synthetic Construct
  source 1..20: mol_type = other DNA
caggcagttgagtggtgtca

SEQ ID NO: 292 - DNA, 18 bp, synthetic construct
  misc_feature 1..18: note = Synthetic Construct
  source 1..18: mol_type = other DNA
aggcagttgagtggtgtc

SEQ ID NO: 293 - DNA, 19 bp, synthetic construct
  misc_feature 1..19: note = Synthetic Construct
  source 1..19: mol_type = other DNA
caggcagttgagtggtgtc

SEQ ID NO: 294 - DNA, 20 bp, synthetic construct
  misc_feature 1..20: note = Synthetic Construct
  source 1..20: mol_type = other DNA
ccaggcagttgagtggtgtc

SEQ ID NO: 295 - DNA, 18 bp, synthetic construct
  misc_feature 1..18: note = Synthetic Construct
  source 1..18: mol_type = other DNA
caggcagttgagtggtgt

SEQ ID NO: 296 - DNA, 19 bp, synthetic construct
  misc_feature 1..19: note = Synthetic Construct
  source 1..19: mol_type = other DNA
ccaggcagttgagtggtgt

SEQ ID NO: 297 - DNA, 20 bp, synthetic construct
  misc_feature 1..20: note = Synthetic Construct
  source 1..20: mol_type = other DNA
gccaggcagttgagtggtgt

SEQ ID NO: 298 - DNA, 20 bp, synthetic construct
  misc_feature 1..20: note = Synthetic Construct
  source 1..20: mol_type = other DNA
tgccaggcagttgagtggtg

SEQ ID NO: 299 - DNA, 18 bp, synthetic construct
  misc_feature 1..18: note = Synthetic Construct
  source 1..18: mol_type = other DNA
actggatgccacattttc

SEQ ID NO: 300 - DNA, 18 bp, synthetic construct
  misc_feature 1..18: note = Synthetic Construct
  source 1..18: mol_type = other DNA
gactggatgccacatttt

SEQ ID NO: 301 - DNA, 20 bp, synthetic construct
  misc_feature 1..20: note = Synthetic Construct
  source 1..20: mol_type = other DNA
tggtaaagtggactggatgc

SEQ ID NO: 302 - DNA, 18 bp, synthetic construct
  misc_feature 1..18: note = Synthetic Construct
  source 1..18: mol_type = other DNA
ggtaaagtggactggatg

SEQ ID NO: 303 - DNA, 19 bp, synthetic construct
  misc_feature 1..19: note = Synthetic Construct
  source 1..19: mol_type = other DNA
tggtaaagtggactggatg

SEQ ID NO: 304 - DNA, 20 bp, synthetic construct
  misc_feature 1..20: note = Synthetic Construct
  source 1..20: mol_type = other DNA
atggtaaagtggactggatg

SEQ ID NO: 305 - DNA, 18 bp, synthetic construct
  misc_feature 1..18: note = Synthetic Construct
  source 1..18: mol_type = other DNA
tggtaaagtggactggat

SEQ ID NO: 306 - DNA, 19 bp, synthetic construct
  misc_feature 1..19: note = Synthetic Construct
  source 1..19: mol_type = other DNA
atggtaaagtggactggat

SEQ ID NO: 307 - DNA, 20 bp, synthetic construct
  misc_feature 1..20: note = Synthetic Construct
  source 1..20: mol_type = other DNA
gatggtaaagtggactggat

SEQ ID NO: 308 - DNA, 20 bp, synthetic construct
  misc_feature 1..20: note = Synthetic Construct
  source 1..20: mol_type = other DNA
cagagatggtttccttaaac

SEQ ID NO: 309 - DNA, 20 bp, synthetic construct
  misc_feature 1..20: note = Synthetic Construct
  source 1..20: mol_type = other DNA
ccagagatggtttccttaaa

SEQ ID NO: 310 - DNA, 19 bp, synthetic construct
  misc_feature 1..19: note = Synthetic Construct
  source 1..19: mol_type = other DNA
ccagagatggtttccttaa

SEQ ID NO: 311 - DNA, 18 bp, synthetic construct
  misc_feature 1..18: note = Synthetic Construct
  source 1..18: mol_type = other DNA
ccagagatggtttcctta

SEQ ID NO: 312 - RNA, 19 nt, synthetic construct
  misc_feature 1..19: note = Synthetic Construct
  source 1..19: mol_type = other RNA
ataaggatgactgaggaag

SEQ ID NO: 313 - RNA, 20 nt, synthetic construct
  misc_feature 1..20: note = Synthetic Construct
  source 1..20: mol_type = other RNA
ataaggatgactgaggaaga

SEQ ID NO: 314 - RNA, 18 nt, synthetic construct
  misc_feature 1..18: note = Synthetic Construct
  source 1..18: mol_type = other RNA
taaggatgactgaggaag

SEQ ID NO: 315 - RNA, 19 nt, synthetic construct
  misc_feature 1..19: note = Synthetic Construct
  source 1..19: mol_type = other RNA
taaggatgactgaggaaga

SEQ ID NO: 316 - RNA, 20 nt, synthetic construct
  misc_feature 1..20: note = Synthetic Construct
  source 1..20: mol_type = other RNA
taaggatgactgaggaagag

SEQ ID NO: 317 - RNA, 18 nt, synthetic construct
  misc_feature 1..18: note = Synthetic Construct
  source 1..18: mol_type = other RNA
aaggatgactgaggaaga

SEQ ID NO: 318 - RNA, 19 nt, synthetic construct
  misc_feature 1..19: note = Synthetic Construct
  source 1..19: mol_type = other RNA
aaggatgactgaggaagag

SEQ ID NO: 319 - RNA, 20 nt, synthetic construct
  misc_feature 1..20: note = Synthetic Construct
  source 1..20: mol_type = other RNA
aaggatgactgaggaagagt

SEQ ID NO: 320 - RNA, 18 nt, synthetic construct
  misc_feature 1..18: note = Synthetic Construct
  source 1..18: mol_type = other RNA
aggatgactgaggaagag

SEQ ID NO: 321 - RNA, 19 nt, synthetic construct
  misc_feature 1..19: note = Synthetic Construct
  source 1..19: mol_type = other RNA
aggatgactgaggaagagt

SEQ ID NO: 322 - RNA, 20 nt, synthetic construct
  misc_feature 1..20: note = Synthetic Construct
  source 1..20: mol_type = other RNA
aggatgactgaggaagagta

SEQ ID NO: 323 - RNA, 18 nt, synthetic construct
  misc_feature 1..18: note = Synthetic Construct
  source 1..18: mol_type = other RNA
ggatgactgaggaagagt

SEQ ID NO: 324 - RNA, 19 nt, synthetic construct
  misc_feature 1..19: note = Synthetic Construct
  source 1..19: mol_type = other RNA
ggatgactgaggaagagta

SEQ ID NO: 325 - RNA, 20 nt, synthetic construct
  misc_feature 1..20: note = Synthetic Construct
  source 1..20: mol_type = other RNA
ggatgactgaggaagagtac

SEQ ID NO: 326 - RNA, 18 nt, synthetic construct
  misc_feature 1..18: note = Synthetic Construct
  source 1..18: mol_type = other RNA
gatgactgaggaagagta

SEQ ID NO: 327 - RNA, 19 nt, synthetic construct
  misc_feature 1..19: note = Synthetic Construct
  source 1..19: mol_type = other RNA
gatgactgaggaagagtac

SEQ ID NO: 328 - RNA, 20 nt, synthetic construct
  misc_feature 1..20: note = Synthetic Construct
  source 1..20: mol_type = other RNA
gatgactgaggaagagtact

SEQ ID NO: 329 - RNA, 18 nt, synthetic construct
  misc_feature 1..18: note = Synthetic Construct
  source 1..18: mol_type = other RNA
atgactgaggaagagtac

SEQ ID NO: 330 - RNA, 19 nt, synthetic construct
  misc_feature 1..19: note = Synthetic Construct
  source 1..19: mol_type = other RNA
atgactgaggaagagtact

SEQ ID NO: 331 - RNA, 20 nt, synthetic construct
  misc_feature 1..20: note = Synthetic Construct
  source 1..20: mol_type = other RNA
atgactgaggaagagtactc

SEQ ID NO: 332 - RNA, 18 nt, synthetic construct
  misc_feature 1..18: note = Synthetic Construct
  source 1..18: mol_type = other RNA
tgactgaggaagagtact

SEQ ID NO: 333 - RNA, 19 nt, synthetic construct
  misc_feature 1..19: note = Synthetic Construct
  source 1..19: mol_type = other RNA
tgactgaggaagagtactc

SEQ ID NO: 334 - RNA, 20 nt, synthetic construct
  misc_feature 1..20: note = Synthetic Construct
  source 1..20: mol_type = other RNA
tgactgaggaagagtactct

SEQ ID NO: 335 - DNA, 19 bp, synthetic construct
  misc_feature 1..19: note = Synthetic Construct
  source 1..19: mol_type = other DNA
cttcctcagtcatccttat

SEQ ID NO: 336 - DNA, 20 bp, synthetic construct
  misc_feature 1..20: note = Synthetic Construct
  source 1..20: mol_type = other DNA
tcttcctcagtcatccttat

SEQ ID NO: 337 - DNA, 18 bp, synthetic construct
  misc_feature 1..18: note = Synthetic Construct
  source 1..18: mol_type = other DNA
cttcctcagtcatcctta

SEQ ID NO: 338 - DNA, 19 bp, synthetic construct
  misc_feature 1..19: note = Synthetic Construct
  source 1..19: mol_type = other DNA
tcttcctcagtcatcctta

SEQ ID NO: 339 - DNA, 20 bp, synthetic construct
  misc_feature 1..20: note = Synthetic Construct
  source 1..20: mol_type = other DNA
ctcttcctcagtcatcctta

SEQ ID NO: 340 - DNA, 18 bp, synthetic construct
  misc_feature 1..18: note = Synthetic Construct
  source 1..18: mol_type = other DNA
tcttcctcagtcatcctt

SEQ ID NO: 341 - DNA, 19 bp, synthetic construct
  misc_feature 1..19: note = Synthetic Construct
  source 1..19: mol_type = other DNA
ctcttcctcagtcatcctt

SEQ ID NO: 342 - DNA, 20 bp, synthetic construct
  misc_feature 1..20: note = Synthetic Construct
  source 1..20: mol_type = other DNA
actcttcctcagtcatcctt

SEQ ID NO: 343 - DNA, 18 bp, synthetic construct
  misc_feature 1..18: note = Synthetic Construct
  source 1..18: mol_type = other DNA
ctcttcctcagtcatcct

SEQ ID NO: 344 - DNA, 19 bp, synthetic construct
  misc_feature 1..19: note = Synthetic Construct
  source 1..19: mol_type = other DNA
actcttcctcagtcatcct

SEQ ID NO: 345 - DNA, 20 bp, synthetic construct
  misc_feature 1..20: note = Synthetic Construct
  source 1..20: mol_type = other DNA
tactcttcctcagtcatcct

SEQ ID NO: 346 - DNA, 18 bp, synthetic construct
  misc_feature 1..18: note = Synthetic Construct
  source 1..18: mol_type = other DNA
actcttcctcagtcatcc

SEQ ID NO: 347 - DNA, 19 bp, synthetic construct
  misc_feature 1..19: note = Synthetic Construct
  source 1..19: mol_type = other DNA
tactcttcctcagtcatcc

SEQ ID NO: 348 - DNA, 20 bp, synthetic construct
  misc_feature 1..20: note = Synthetic Construct
  source 1..20: mol_type = other DNA
gtactcttcctcagtcatcc

SEQ ID NO: 349 - DNA, 18 bp, synthetic construct
  misc_feature 1..18: note = Synthetic Construct
  source 1..18: mol_type = other DNA
tactcttcctcagtcatc

SEQ ID NO: 350 - DNA, 19 bp, synthetic construct
  misc_feature 1..19: note = Synthetic Construct
  source 1..19: mol_type = other DNA
gtactcttcctcagtcatc

SEQ ID NO: 351 - DNA, 20 bp, synthetic construct
  misc_feature 1..20: note = Synthetic Construct
  source 1..20: mol_type = other DNA
agtactcttcctcagtcatc

SEQ ID NO: 352 - DNA, 18 bp, synthetic construct
  misc_feature 1..18: note = Synthetic Construct
  source 1..18: mol_type = other DNA
gtactcttcctcagtcat

SEQ ID NO: 353 - DNA, 19 bp, synthetic construct
  misc_feature 1..19: note = Synthetic Construct
  source 1..19: mol_type = other DNA
agtactcttcctcagtcat

SEQ ID NO: 354 - DNA, 20 bp, synthetic construct
  misc_feature 1..20: note = Synthetic Construct
  source 1..20: mol_type = other DNA
gagtactcttcctcagtcat

SEQ ID NO: 355 - DNA, 18 bp, synthetic construct
  misc_feature 1..18: note = Synthetic Construct
  source 1..18: mol_type = other DNA
agtactcttcctcagtca

SEQ ID NO: 356 - DNA, 19 bp, synthetic construct
  misc_feature 1..19: note = Synthetic Construct
  source 1..19: mol_type = other DNA
gagtactcttcctcagtca

SEQ ID NO: 357 - DNA, 20 bp, synthetic construct
  misc_feature 1..20: note = Synthetic Construct
  source 1..20: mol_type = other DNA
agagtactcttcctcagtca

SEQ ID NO: 358 - DNA, 20 bp, synthetic construct
  misc_feature 1..20: note = Synthetic Construct
  misc_feature 1..20: note = Description of Combined DNA/RNA Molecule: Synthetic oligonucleotide
  modified_base 1..2: mod_base = cm
  misc_feature 1..20: note = phosphorothioate backbone
  modified_base 3: mod_base = OTHER; note = 2'-O-methyladenosine
  modified_base 4: mod_base = OTHER; note = 2'-O-methylguanosine
  modified_base 5: mod_base = cm; note = 2'-O-methylcytidine
  modified_base 16: mod_base = OTHER; note = 2'-O-methyladenosine
  modified_base 17: mod_base = um; note = 2'-O-methyluridine
  modified_base 18: mod_base = cm; note = 2'-O-methylcytidine
  modified_base 19: mod_base = OTHER; note = 2'-O-methyladenosine
  modified_base 20: mod_base = um
  source 1..20: mol_type = other DNA
nnnnncttgttggatnnnnn

SEQ ID NO: 359 - DNA, 20 bp, synthetic construct
  misc_feature 1..20: note = Synthetic Construct
  misc_feature 1..20: note = Description of Combined DNA/RNA Molecule: Synthetic oligonucleotide
  modified_base 1..2: mod_base = OTHER; note = 2'-O-methylcytidine
  misc_feature 1..20: note = phosphorothioate backbone
  modified_base 3: mod_base = OTHER; note = 2'-O-methyladenosine
  modified_base 4: mod_base = OTHER; note = 2'-O-methylcytidine
  modified_base 5: mod_base = OTHER; note = 2'-O-methyladenosine
  modified_base 16: mod_base = OTHER; note = 2'-O-methyluridine
  modified_base 17..18: mod_base = OTHER; note = 2'-O-methylguanosine
  modified_base 19..20: mod_base = OTHER; note = 2'-O-methyladenosine
  source 1..20: mol_type = other DNA
nnnnntttcctctcannnnn

SEQ ID NO: 360 - DNA, 20 bp, synthetic construct
  misc_feature 1..20: note = Synthetic Construct
  misc_feature 1..20: note = Description of Combined DNA/RNA Molecule: Synthetic oligonucleotide
  misc_feature 1..20: note = phosphorothioate backbone
  modified_base 1: mod_base = OTHER; note = 2'-O-methylguanosine
  modified_base 2: mod_base = OTHER; note = 2'-O-methyladenosine
  modified_base 3: mod_base = OTHER; note = 2'-O-methylguanosine
  modified_base 4: mod_base = OTHER; note = 2'-O-methyluridine
  modified_base 5: mod_base = OTHER; note = 2'-O-methylguanosine
  modified_base 16..17: mod_base = OTHER; note = 2'-O-methyladenosine
  modified_base 18: mod_base = OTHER; note = 2'-O-methyluridine
  modified_base 19: mod_base = OTHER; note = 2'-O-methylguanosine
  modified_base 20: mod_base = OTHER; note = 2'-O-methyluridine
  source 1..20: mol_type = other DNA
nnnnntttgcaaaccnnnnn

SEQ ID NO: 361 - DNA, 20 bp, synthetic construct
  misc_feature 1..20: note = Synthetic Construct
  misc_feature 1..20: note = Description of Combined DNA/RNA Molecule: Synthetic oligonucleotide
  modified_base 1: mod_base = OTHER; note = 2'-O-methyluridine
  misc_feature 1..20: note = phosphorothioate backbone
  modified_base 2: mod_base = OTHER; note = 2'-O-methylguanosine
  modified_base 3..5: mod_base = OTHER; note = 2'-O-methyluridine
  modified_base 16: mod_base = OTHER; note = 2'-O-methyluridine
  modified_base 17: mod_base = OTHER; note = 2'-O-methylcytidine
  modified_base 18: mod_base = OTHER; note = 2'-O-methyluridine
  modified_base 19: mod_base = OTHER; note = 2'-O-methylguanosine
  modified_base 20: mod_base = OTHER; note = 2'-O-methylcytidine
  source 1..20: mol_type = other DNA
nnnnnctttggtgatnnnnn

SEQ ID NO: 362 - DNA, 20 bp, synthetic construct
  misc_feature 1..20: note = Synthetic Construct
  misc_feature 1..20: note = Description of Combined DNA/RNA Molecule: Synthetic oligonucleotide
  modified_base 1: mod_base = OTHER; note = 2'-O-methyluridine
  misc_feature 1..20: note = phosphorothioate backbone
  modified_base 2: mod_base = OTHER; note = 2'-O-methyladenosine
  modified_base 3: mod_base = OTHER; note = 2'-O-methylguanosine
  modified_base 4: mod_base = OTHER; note = 2'-O-methyladenosine
  modified_base 5: mod_base = OTHER; note = 2'-O-methylguanosine
  modified_base 16..17: mod_base = OTHER; note = 2'-O-methylguanosine
  modified_base 18: mod_base = OTHER; note = 2'-O-methylcytidine
  modified_base 19: mod_base = OTHER; note = 2'-O-methyladenosine
  modified_base 20: mod_base = OTHER; note = 2'-O-methylcytidine
  source 1..20: mol_type = other DNA
nnnnngtgaaggccannnnn

SEQ ID NO: 363 - DNA, 20 bp, synthetic construct
  misc_feature 1..20: note = Synthetic Construct
  misc_feature 1..20: note = Description of Combined DNA/RNA Molecule: Synthetic oligonucleotide
  modified_base 1: mod_base = OTHER; note = 2'-O-methylguanosine
  misc_feature 1..20: note = phosphorothioate backbone
  modified_base 2: mod_base = OTHER; note = 2'-O-methyluridine
  modified_base 3: mod_base = OTHER; note = 2'-O-methyladenosine
  modified_base 4: mod_base = OTHER; note = 2'-O-methylcytidine
  modified_base 5: mod_base = OTHER; note = 2'-O-methyluridine
  modified_base 16: mod_base = OTHER; note = 2'-O-methylcytidine
  modified_base 17: mod_base = OTHER; note = 2'-O-methyladenosine
  modified_base 18: mod_base = OTHER; note = 2'-O-methyluridine
  modified_base 19..20: mod_base = OTHER; note = 2'-O-methylcytidine
  source 1..20: mol_type = other DNA
nnnnncttcctcagtnnnnn

SEQ ID NO: 364 - DNA, 20 bp, synthetic construct
  misc_feature 1..20: note = Synthetic Construct
  misc_feature 1..20: note = Description of Combined DNA/RNA Molecule: Synthetic oligonucleotide
  modified_base 1: mod_base = OTHER; note = 2'-O-methyluridine
  misc_feature 1..20: note = phosphorothioate backbone
  modified_base 2: mod_base = OTHER; note = 2'-O-methylguanosine
  modified_base 3: mod_base = OTHER; note = 2'-O-methyluridine
  modified_base 4: mod_base = OTHER; note = 2'-O-methylcytidine
  modified_base 5: mod_base = OTHER; note = 2'-O-methyladenosine
  modified_base 16: mod_base = OTHER; note = 2'-O-methylguanosine
  modified_base 17..18: mod_base = OTHER; note = 2'-O-methyladenosine
  modified_base 19: mod_base = OTHER; note = 2'-O-methylcytidine
  modified_base 20: mod_base = OTHER; note = 2'-O-methyladenosine
  source 1..20: mol_type = other DNA
nnnnngtttctccctnnnnn

SEQ ID NO: 365 - DNA, 20 bp, synthetic construct
  misc_feature 1..20: note = Synthetic Construct
  misc_feature 1..20: note = Description of Combined DNA/RNA Molecule: Synthetic oligonucleotide
  modified_base 1: mod_base = OTHER; note = 2'-O-methyluridine
  misc_feature 1..20: note = phosphorothioate backbone
  modified_base 2: mod_base = OTHER; note = 2'-O-methyladenosine
  modified_base 3: mod_base = OTHER; note = 2'-O-methylguanosine
  modified_base 4..5: mod_base = OTHER; note = 2'-O-methyladenosine
  modified_base 16: mod_base = OTHER; note = 2'-O-methylcytidine
  modified_base 17..18: mod_base = OTHER; note = 2'-O-methyluridine
  modified_base 19..20: mod_base = OTHER; note = 2'-O-methylguanosine
  source 1..20: mol_type = other DNA
nnnnntggcacatctnnnnn

SEQ ID NO: 366 - DNA, 20 bp, synthetic construct
  misc_feature 1..20: note = Synthetic Construct
  misc_feature 1..20: note = Description of Combined DNA/RNA Molecule: Synthetic oligonucleotide
  modified_base 1: mod_base = OTHER; note = 2'-O-methylguanosine
  misc_feature 1..20: note = phosphorothioate backbone
  modified_base 2..5: mod_base = OTHER; note = 2'-O-methyluridine
  modified_base 16: mod_base = OTHER; note = 2'-O-methyladenosine
  modified_base 17: mod_base = OTHER; note = 2'-O-methylguanosine
  modified_base 18: mod_base = OTHER; note = 2'-O-methyluridine
  modified_base 19: mod_base = OTHER; note = 2'-O-methylcytidine
  modified_base 20: mod_base = OTHER; note = 2'-O-methyluridine
  source 1..20: mol_type = other DNA
nnnnncttcctccacnnnnn

SEQ ID NO: 367 - DNA, 20 bp, synthetic construct
  misc_feature 1..20: note = Synthetic Construct
  misc_feature 1..20: note = Description of Combined DNA/RNA Molecule: Synthetic oligonucleotide
  modified_base 1: mod_base = OTHER; note = 2'-O-methylcytidine
  misc_feature 1..20: note = phosphorothioate backbone
  modified_base 2: mod_base = OTHER; note = 2'-O-methyluridine
  modified_base 3..4: mod_base = OTHER; note = 2'-O-methylguanosine
  modified_base 5: mod_base = OTHER; note = 2'-O-methyluridine
  modified_base 16: mod_base = OTHER; note = 2'-O-methylcytidine
  modified_base 17..19: mod_base = OTHER; note = 2'-O-methyladenosine
  modified_base 20: mod_base = OTHER; note = 2'-O-methylguanosine
  source 1..20: mol_type = other DNA
nnnnngtcaacaagcnnnnn

SEQ ID NO: 368 - DNA, 19 bp, synthetic construct
  misc_feature 1..19: note = Synthetic Construct
  misc_feature 1..19: note = Description of Combined DNA/RNA Molecule: Synthetic oligonucleotide
  modified_base 1: mod_base = OTHER; note = 2'-O-methylguanosine
  misc_feature 1..19: note = phosphorothioate backbone
  modified_base 2..3: mod_base = OTHER; note = 2'-O-methyluridine
  modified_base 4: mod_base = OTHER; note = 2'-O-methylguanosine
  modified_base 15: mod_base = OTHER; note = 2'-O-methylguanosine
  modified_base 16..18: mod_base = OTHER; note = 2'-O-methyluridine
  modified_base 19: mod_base = OTHER; note = 2'-O-methylcytidine
  source 1..19: mol_type = other DNA
nnnnagtggtgtcannnnn

SEQ ID NO: 369 - DNA, 18 bp, synthetic construct
  misc_feature 1..18: note = Synthetic Construct
  misc_feature 1..18: note = Description of Combined DNA/RNA Molecule: Synthetic oligonucleotide
  modified_base 1..2: mod_base = OTHER; note = 2'-O-methyluridine
  misc_feature 1..18: note = phosphorothioate backbone
  modified_base 3: mod_base = OTHER; note = 2'-O-methylguanosine
  modified_base 4: mod_base = OTHER; note = 2'-O-methyladenosine
  modified_base 15..17: mod_base = OTHER; note = 2'-O-methyluridine
  modified_base 18: mod_base = OTHER; note = 2'-O-methylcytidine
  source 1..18: mol_type = other DNA
nnnngtggtgtcagnnnn

SEQ ID NO: 370 - DNA, 18 bp, synthetic construct
  misc_feature 1..18: note = Synthetic Construct
  misc_feature 1..18: note = Description of Combined DNA/RNA Molecule: Synthetic oligonucleotide
  modified_base 1: mod_base = OTHER; note = 2'-O-methylcytidine
  modified_base 1..18: mod_base = OTHER; note = phosphorothioate backbone
  modified_base 2: mod_base = OTHER; note = 2'-O-methyluridine
  modified_base 3..4: mod_base = OTHER; note = 2'-O-methylguanosine
  modified_base 15..16: mod_base = OTHER; note = 2'-O-methylcytidine
  modified_base 17..18: mod_base = OTHER; note = 2'-O-methyladenosine
  source 1..18: mol_type = other DNA
nnnntgtcaacaagnnnn

SEQ ID NO: 371 - DNA, 20 bp, synthetic construct
  misc_feature 1..20: note = Synthetic Construct
  misc_feature 1..20: note = Description of Combined DNA/RNA Molecule: Synthetic oligonucleotide
  modified_base 1: mod_base = OTHER; note = 2'-O-methyladenosine
  misc_feature 1..20: note = phosphorothioate backbone
  modified_base 2: mod_base = OTHER; note = 2'-O-methyluridine
  modified_base 3: mod_base = OTHER; note = 2'-O-methyladenosine
  modified_base 4: mod_base = OTHER; note = 2'-O-methylguanosine
  modified_base 5: mod_base = OTHER; note = 2'-O-methyladenosine
  modified_base 16: mod_base = OTHER; note = 2'-O-methyluridine
  modified_base 17: mod_base = OTHER; note = 2'-O-methylcytidine
  modified_base 18..19: mod_base = OTHER; note = 2'-O-methyluridine
  modified_base 20: mod_base = OTHER; note = 2'-O-methylguanosine
  source 1..20: mol_type = other DNA
nnnnnatggcacatcnnnnn

SEQ ID NO: 372 - DNA, 19 bp, synthetic construct
  misc_feature 1..19: note = Synthetic Construct
  misc_feature 1..19: note = Description of Combined DNA/RNA Molecule: Synthetic oligonucleotide
  modified_base 1: mod_base = OTHER; note = 2'-O-methyladenosine
  misc_feature 1..19: note = phosphorothioate backbone
  modified_base 2: mod_base = OTHER; note = 2'-O-methylguanosine
  modified_base 3..4: mod_base = OTHER; note = 2'-O-methyladenosine
  modified_base 15: mod_base = OTHER; note = 2'-O-methylcytidine
  modified_base 16..17: mod_base = OTHER; note = 2'-O-methyluridine
  modified_base 18..19: mod_base = OTHER; note = 2'-O-methylguanosine
  source 1..19: mol_type = other DNA
nnnntggcacatctnnnnn

SEQ ID NO: 373 - DNA, 19 bp, synthetic construct
  misc_feature 1..19: note = Synthetic Construct
  misc_feature 1..19: note = Description of Combined DNA/RNA Molecule: Synthetic oligonucleotide
  modified_base 1: mod_base = OTHER; note = 2'-O-methyluridine
  misc_feature 1..19: note = phosphorothioate backbone
  modified_base 2: mod_base = OTHER; note = 2'-O-methyladenosine
  modified_base 3: mod_base = OTHER; note = 2'-O-methylguanosine
  modified_base 4: mod_base = OTHER; note = 2'-O-methyladenosine
  modified_base 15: mod_base = OTHER; note = 2'-O-methyluridine
  modified_base 16: mod_base = OTHER; note = 2'-O-methylcytidine
  modified_base 17..18: mod_base = OTHER; note = 2'-O-methyluridine
  modified_base 19: mod_base = OTHER; note = 2'-O-methylguanosine
  source 1..19: mol_type = other DNA
nnnnatggcacatcnnnnn

SEQ ID NO: 374 - DNA, 18 bp, synthetic construct
  misc_feature 1..18: note = Synthetic Construct
  misc_feature 1..18: note = Description of Combined DNA/RNA Molecule: Synthetic oligonucleotide
  modified_base 1: mod_base = OTHER; note = 2'-O-methyladenosine
  misc_feature 1..18: note = phosphorothioate backbone
  modified_base 2: mod_base = OTHER; note = 2'-O-methylguanosine
  modified_base 3..4: mod_base = OTHER; note = 2'-O-methyladenosine
  modified_base 15: mod_base = OTHER; note = 2'-O-methylcytidine
  modified_base 16..17: mod_base = OTHER; note = 2'-O-methyluridine
  modified_base 18: mod_base = OTHER; note = 2'-O-methylguanosine
  source 1..18: mol_type = other DNA
nnnntggcacatctnnnn

SEQ ID NO: 375 - DNA, 20 bp, synthetic construct
  misc_feature 1..20: note = Synthetic Construct
  misc_feature 1..20: note = Description of Combined DNA/RNA Molecule: Synthetic oligonucleotide
  modified_base 1: mod_base = OTHER; note = 2'-O-methyluridine
  misc_feature 1..20: note = phosphorothioate backbone
  modified_base 2: mod_base = OTHER; note = 2'-O-methyladenosine
  modified_base 3: mod_base = OTHER; note = 2'-O-methylguanosine
  modified_base 4..5: mod_base = OTHER; note = 2'-O-methyladenosine
  modified_base 16: mod_base = OTHER; note = 2'-O-methylcytidine
  modified_base 17..18: mod_base = OTHER; note = 2'-O-methyluridine
  modified_base 19..20: mod_base = OTHER; note = 2'-O-methylguanosine
  source 1..20: mol_type = other DNA
nnnnntggcacatctnnnnn

SEQ ID NO: 376 - DNA, 20 bp, synthetic construct
  misc_feature 1..20: note = Synthetic Construct
  misc_feature 1..20: note = Description of Combined DNA/RNA Molecule: Synthetic oligonucleotide
  modified_base 1: mod_base = OTHER; note = 2'-O-methyluridine
  misc_feature 1..5: note = phosphorothioate backbone
  modified_base 2: mod_base = OTHER; note = 2'-O-methyladenosine
  modified_base 3: mod_base = OTHER; note = 2'-O-methylguanosine
  modified_base 4..5: mod_base = OTHER; note = 2'-O-methyladenosine
  misc_feature 5..6: note = phosphodiester backbone
  misc_feature 6..15: note = phosphorothioate backbone
  misc_feature 15..16: note = phosphodiester backbone
  misc_feature 16..20: note = phosphorothioate backbone
  modified_base 16: mod_base = OTHER; note = 2'-O-methylcytidine
  modified_base 17..18: mod_base = OTHER; note = 2'-O-methyluridine
  modified_base 19..20: mod_base = OTHER; note = 2'-O-methylguanosine
  source 1..20: mol_type = other DNA
nnnnntggcacatctnnnnn

SEQ ID NO: 377 - DNA, 20 bp, synthetic construct
  misc_feature 1..20: note = Synthetic Construct
  misc_feature 1..20: note = Description of Combined DNA/RNA Molecule: Synthetic oligonucleotide
  modified_base 1: mod_base = OTHER; note = 2'-O-methyluridine
  misc_feature 1..2: note = phosphorothioate backbone
  modified_base 2: mod_base = OTHER; note = 2'-O-methyladenosine
  misc_feature 2..3: note = phosphodiester backbone
  modified_base 3: mod_base = OTHER; note = 2'-O-methylguanosine
  misc_feature 3..4: note = phosphorothioate backbone
  misc_feature 4..5: note = phosphodiester backbone
  modified_base 4..5: mod_base = OTHER; note = 2'-O-methyladenosine
  misc_feature 5..6: note = phosphorothioate backbone
  misc_feature 6..7: note = phosphodiester backbone
  misc_feature 7..8: note = phosphorothioate backbone
  misc_feature 8..9: note = phosphodiester backbone
  misc_feature 9..10: note = phosphorothioate backbone
  misc_feature 10..11: note = phosphodiester backbone
  misc_feature 11..12: note = phosphorothioate backbone
  misc_feature 12..13: note = phosphodiester backbone
  misc_feature 13..14: note = phosphorothioate backbone
  misc_feature 14..15: note = phosphodiester backbone
  misc_feature 15..16: note = phosphorothioate backbone
  modified_base 16: mod_base = OTHER; note = 2'-O-methylcytidine
  misc_feature 17..18: note = phosphorothioate backbone
  modified_base 17..18: mod_base = OTHER; note = 2'-O-methyluridine
  misc_feature 18..19: note = phosphodiester backbone
  misc_feature 19..20: note = phosphorothioate backbone
  modified_base 19..20: mod_base = OTHER; note = 2'-O-methylguanosine
  source 1..20: mol_type = other DNA
nnnnntggcacatctnnnnn

SEQ ID NO: 378 - DNA, 20 bp, synthetic construct
  misc_feature 1..20: note = Synthetic Construct
  misc_feature 1..20: note = Description of Combined DNA/RNA Molecule: Synthetic oligonucleotide
  modified_base 1: mod_base = OTHER; note = 2'-O-(2-methoxyethyl)-modified thymidine
  misc_feature 1..20: note = phosphorothioate backbone
  modified_base 2: mod_base = OTHER; note = 2'-O-(2-methoxyethyl)-modified adenosine
  modified_base 3: mod_base = OTHER; note = 2'-O-(2-methoxyethyl)-modified guanosine
  modified_base 4..5: mod_base = OTHER; note = 2'-O-(2-methoxyethyl)-modified adenosine
  modified_base 16: mod_base = OTHER; note = 2'-O-(2-methoxyethyl)-modified 5-methylcytidine
  modified_base 17..18: mod_base = OTHER; note = 2'-O-(2-methoxyethyl)-modified thymidine
  modified_base 19..20: mod_base = OTHER; note = 2'-O-(2-methoxyethyl)-modified guanosine
  source 1..20: mol_type = other DNA
nnnnntggcacatctnnnnn

SEQ ID NO: 379 - DNA, 20 bp, synthetic construct
  misc_feature 1..20: note = Synthetic Construct
  misc_feature 1..20: note = Description of Combined DNA/RNA Molecule: Synthetic oligonucleotide
  misc_feature 1..5: note = phosphorothioate backbone
  modified_base 1: mod_base = OTHER; note = 2'-O-(2-methoxyethyl)-modified thymidine
  modified_base 2: mod_base = OTHER; note = 2'-O-(2-methoxyethyl)-modified adenosine
  modified_base 3: mod_base = OTHER; note = 2'-O-(2-methoxyethyl)-modified guanosine
  modified_base 4..5: mod_base = OTHER; note = 2'-O-(2-methoxyethyl)-modified adenosine
  misc_feature 5..6: note = phosphodiester backbone
  misc_feature 6..15: note = phosphorothioate backbone
  misc_feature 15..16: note = phosphodiester backbone
  modified_base 16: mod_base = OTHER; note = 2'-O-(2-methoxyethyl)-modified 5-methylcytidine
  misc_feature 16..20: note = phosphorothioate backbone
  modified_base 17..18: mod_base = OTHER; note = 2'-O-(2-methoxyethyl)-modified thymidine
  modified_base 19..20: mod_base = OTHER; note = 2'-O-(2-methoxyethyl)-modified guanosine
  source 1..20: mol_type = other DNA
nnnnntggcacatctnnnnn

SEQ ID NO: 380 - DNA, 20 bp, synthetic construct
  misc_feature 1..20: note = Synthetic Construct
  misc_feature 1..20: note = Description of Combined DNA/RNA Molecule: Synthetic oligonucleotide
  modified_base 1: mod_base = OTHER; note = 2'-O-(2-methoxyethyl)-modified thymidine
  misc_feature 1..2: note = phosphorothioate backbone
  misc_feature 2..3: note = phosphodiester backbone
  modified_base 2: mod_base = OTHER; note = 2'-O-(2-methoxyethyl)-modified adenosine
  misc_feature 3..4: note = phosphorothioate backbone
  modified_base 3: mod_base = OTHER; note = 2'-O-(2-methoxyethyl)-modified guanosine
  misc_feature 4..5: note = phosphodiester backbone
  modified_base 4..5: mod_base = OTHER; note = 2'-O-(2-methoxyethyl)-modified adenosine
  misc_feature 5..6: note = phosphorothioate backbone
  misc_feature 6..7: note = phosphodiester backbone
  misc_feature 7..8: note = phosphorothioate backbone
  misc_feature 8..9: note = phosphodiester backbone
  misc_feature 9..10: note = phosphorothioate backbone
  misc_feature 10..11: note = phosphodiester backbone
  misc_feature 11..12: note = phosphorothioate backbone
  misc_feature 12..13: note = phosphodiester backbone
  misc_feature 13..14: note = phosphorothioate backbone
  misc_feature 14..15: note = phosphodiester backbone
  misc_feature 15..16: note = phosphorothioate backbone
  misc_feature 16..17: note = phosphodiester backbone
  modified_base 16: mod_base = OTHER; note = 2'-O-(2-methoxyethyl)-modified 5-methylcytidine
  misc_feature 17..18: note = phosphorothioate backbone
  modified_base 17..18: mod_base = OTHER; note = 2'-O-(2-methoxyethyl)-modified thymidine
  misc_feature 18..19: note = phosphodiester backbone
  misc_feature 19..20: note = phosphorothioate backbone
  modified_base 19..20: mod_base = OTHER; note = 2'-O-(2-methoxyethyl)-modified guanosine
  source 1..20: mol_type = other DNA
nnnnntggcacatctnnnnn

SEQ ID NO: 381 - DNA, 18 bp, synthetic construct
  misc_feature 1..18: note = Synthetic Construct
  misc_feature 1..18: note = Description of Combined DNA/RNA Molecule: Synthetic oligonucleotide
  modified_base 1: mod_base = OTHER; note = locked nucleic acid adenosine
  misc_feature 1..18: note = phosphorothioate backbone
  modified_base 2: mod_base = OTHER; note = locked nucleic acid guanosine
  modified_base 3: mod_base = OTHER; note = locked nucleic acid adenosine
  modified_base 15: mod_base = OTHER; note = locked nucleic acid 5-methylcytidine
  modified_base 16..17: mod_base = OTHER; note = locked nucleic acid thymidine
  modified_base 18: mod_base = OTHER; note = locked nucleic acid guanosine
  source 1..18: mol_type = other DNA
nnnatggcacatctnnnn

SEQ ID NO: 382 - DNA, 18 bp, synthetic construct
  misc_feature 1..18: note = Synthetic Construct
  misc_feature 1..18: note = Description of Combined DNA/RNA Molecule: Synthetic oligonucleotide
  modified_base 1: mod_base = OTHER; note = locked nucleic acid adenosine
  misc_feature 1..3: note = phosphorothioate backbone
  modified_base 2: mod_base = OTHER; note = locked nucleic acid guanosine
  misc_feature 3..4: note = phosphodiester backbone
  modified_base 3: mod_base = OTHER; note = locked nucleic acid adenosine
  misc_feature 4..14: note = phosphorothioate backbone
  misc_feature 14..15: note = phosphodiester backbone
  misc_feature 15..18: note = phosphorothioate backbone
  modified_base 15: mod_base = OTHER; note = locked nucleic acid 5-methylcytidine
  modified_base 16..17: mod_base = OTHER; note = locked nucleic acid thymidine
  modified_base 18: mod_base = OTHER; note = locked nucleic acid guanosine
  source 1..18: mol_type = other DNA
nnnatggcacatctnnnn

SEQ ID NO: 383 - DNA, 18 bp, synthetic construct
  misc_feature 1..18: note = Synthetic Construct
  misc_feature 1..18: note = Description of Combined DNA/RNA Molecule: Synthetic oligonucleotide
  modified_base 1: mod_base = OTHER; note = locked nucleic acid adenosine
  misc_feature 1..2: note = phosphorothioate backbone
  misc_feature 2..3: note = phosphodiester backbone
  modified_base 2: mod_base = OTHER; note = locked nucleic acid guanosine
  misc_feature 3..4: note = phosphorothioate backbone
  modified_base 3: mod_base = OTHER; note = locked nucleic acid adenosine
  misc_feature 4..5: note = phosphodiester backbone
  misc_feature 5..6: note = phosphorothioate backbone
  misc_feature 6..7: note = phosphodiester backbone
  misc_feature 7..8: note = phosphorothioate backbone
  misc_feature 8..9: note = phosphodiester backbone
  misc_feature 9..10: note = phosphorothioate backbone
  misc_feature 10..11: note = phosphodiester backbone
  misc_feature 11..12: note = phosphorothioate backbone
  misc_feature 12..13: note = phosphodiester backbone
  misc_feature 13..14: note = phosphorothioate backbone
  misc_feature 14..15: note = phosphodiester backbone
  misc_feature 15..16: note = phosphorothioate backbone
  modified_base 15: mod_base = OTHER; note = locked nucleic acid 5-methylcytidine
  misc_feature 16..17: note = phosphodiester backbone
  modified_base 16..17: mod_base = OTHER; note = locked nucleic acid thymidine
  misc_feature 17..18: note = phosphorothioate backbone
  modified_base 18: mod_base = OTHER; note = locked nucleic acid guanosine
  source 1..18: mol_type = other DNA
nnnatggcacatctnnnn

SEQ ID NO: 384 - DNA, 18 bp, synthetic construct
  misc_feature 1..18: note = Synthetic Construct
  misc_feature 1..18: note = Description of Combined DNA/RNA Molecule: Synthetic oligonucleotide
  modified_base 1: mod_base = OTHER; note = 2'-O-methylcytidine
  misc_feature 1..18: note = phosphorothioate backbone
  modified_base 2: mod_base = OTHER; note = 2'-O-methyluridine
  modified_base 3..4: mod_base = OTHER; note = 2'-O-methylguanosine
  modified_base 15..16: mod_base = OTHER; note = 2'-O-methylcytidine
  modified_base 17..18: mod_base = OTHER; note = 2'-O-methyladenosine
  source 1..18: mol_type = other DNA
nnnntgtcaacaagnnnn

SEQ ID NO: 385 - DNA, 18 bp, synthetic construct
  misc_feature 1..18: note = Synthetic Construct
  misc_feature 1..18: note = Description of Combined DNA/RNA Molecule: Synthetic oligonucleotide
  modified_base 1: mod_base = OTHER; note = 2'-O-methylcytidine
  misc_feature 1..4: note = phosphorothioate backbone
  modified_base 2: mod_base = OTHER; note = 2'-O-methyluridine
  modified_base 3..4: mod_base = OTHER; note = 2'-O-methylguanosine
  misc_feature 4..5: note = phosphodiester backbone
  misc_feature 5..14: note = phosphorothioate backbone
  misc_feature 14..15: note = phosphodiester backbone
  misc_feature 15..18: note = phosphorothioate backbone
  modified_base 15..16: mod_base = OTHER; note = 2'-O-methylcytidine
  modified_base 17..18: mod_base = OTHER; note = 2'-O-methyladenosine
  source 1..18: mol_type = other DNA
nnnntgtcaacaagnnnn

SEQ ID NO: 386 - DNA, 18 bp, synthetic construct
  misc_feature 1..18: note = Synthetic Construct
  misc_feature 1..18: note = Description of Combined DNA/RNA Molecule: Synthetic oligonucleotide
  modified_base 1: mod_base = OTHER; note = 2'-O-methylcytidine
  misc_feature 1..2: note = phosphorothioate backbone
  misc_feature 2..3: note = phosphodiester backbone
  modified_base 2: mod_base = OTHER; note = 2'-O-methyluridine
  misc_feature 3..4: note = phosphorothioate backbone
  modified_base 3..4: mod_base = OTHER; note = 2'-O-methylguanosine
  misc_feature 4..5: note = phosphodiester backbone
  misc_feature 5..6: note = phosphorothioate backbone
  misc_feature 6..7: note = phosphodiester backbone
  misc_feature 7..8: note = phosphorothioate backbone
  misc_feature 8..9: note = phosphodiester backbone
  misc_feature 9..10: note = phosphorothioate backbone
  misc_feature 10..11: note = phosphodiester backbone
  misc_feature 11..12: note = phosphorothioate backbone
  misc_feature 12..13: note = phosphodiester backbone
  misc_feature 13..14: note = phosphorothioate backbone
  misc_feature 14..15: note = phosphodiester backbone
  misc_feature 15..16: note = phosphorothioate backbone
  modified_base 15..16: mod_base = OTHER; note = 2'-O-methylcytidine
  misc_feature 16..17: note = phosphodiester backbone
  misc_feature 17..18: note = phosphorothioate backbone
  modified_base 17..18: mod_base = OTHER; note = 2'-O-methyladenosine
  source 1..18: mol_type = other DNA
nnnntgtcaacaagnnnn

SEQ ID NO: 387 - DNA, 18 bp, synthetic construct
  misc_feature 1..18: note = Synthetic Construct
  modified_base 1: mod_base = OTHER; note = 2'-O-(2-methoxyethyl)-modified 5-methylcytidine
  misc_feature 1..18: note = phosphorothioate backbone
  modified_base 2: mod_base = OTHER; note = 2'-O-(2-methoxyethyl)-modified thymidine
  modified_base 3..4: mod_base = OTHER; note = 2'-O-(2-methoxyethyl)-modified guanosine
  modified_base 15..16: mod_base = OTHER; note = 2'-O-(2-methoxyethyl)-modified 5-methylcytidine
  modified_base 17..18: mod_base = OTHER; note = 2'-O-(2-methoxyethyl)-modified adenosine
  source 1..18: mol_type = other DNA
nnnntgtcaacaagnnnn

SEQ ID NO: 388 - DNA, 18 bp, synthetic construct
  misc_feature 1..18: note = Synthetic Construct
  modified_base 1: mod_base = OTHER; note = 2'-O-(2-methoxyethyl)-modified 5-methylcytidine
  misc_feature 1..4: note = phosphorothioate backbone
  modified_base 2: mod_base = OTHER; note = 2'-O-(2-methoxyethyl)-modified thymidine
  modified_base 3..4: mod_base = OTHER; note = 2'-O-(2-methoxyethyl)-modified guanosine
  misc_feature 4..5: note = phosphodiester backbone
  misc_feature 5..14: note = phosphorothioate backbone
  misc_feature 14..15: note = phosphodiester backbone
  misc_feature 15..18: note = phosphorothioate backbone
  modified_base 15..16: mod_base = OTHER; note = 2'-O-(2-methoxyethyl)-modified 5-methylcytidine
  modified_base 17..18: mod_base = OTHER; note = 2'-O-(2-methoxyethyl)-modified adenosine
  source 1..18: mol_type = other DNA
nnnntgtcaacaagnnnn

SEQ ID NO: 389 - DNA, 18 bp, synthetic construct
  misc_feature 1..18: note = Synthetic Construct
  modified_base 1: mod_base = OTHER; note = 2'-O-(2-methoxyethyl)-modified 5-methylcytidine
  misc_feature 1..2: note = phosphorothioate backbone
  misc_feature 2..3: note = phosphodiester backbone
  modified_base 2: mod_base = OTHER; note = 2'-O-(2-methoxyethyl)-modified thymidine
  misc_feature 3..4: note = phosphorothioate backbone
  modified_base 3..4: mod_base = OTHER; note = 2'-O-(2-methoxyethyl)-modified guanosine
  misc_feature 4..5: note = phosphodiester backbone
  misc_feature 5..6: note = phosphorothioate backbone
  misc_feature 6..7: note = phosphodiester backbone
  misc_feature 7..8: note = phosphorothioate backbone
  misc_feature 8..9: note = phosphodiester backbone
  misc_feature 9..10: note = phosphorothioate backbone
  misc_feature 10..11: note = phosphodiester backbone
  misc_feature 11..12: note = phosphorothioate backbone
  misc_feature 12..13: note = phosphodiester backbone
  misc_feature 13..14: note = phosphorothioate backbone
  misc_feature 14..15: note = phosphodiester backbone
  misc_feature 15..16: note = phosphorothioate backbone
  modified_base 15..16: mod_base = OTHER; note = 2'-O-(2-methoxyethyl)-modified 5-methylcytidine
  misc_feature 16..17: note = phosphodiester backbone
  misc_feature 17..18: note = phosphorothioate backbone
  modified_base 17..18: mod_base = OTHER; note = 2'-O-(2-methoxyethyl)-modified adenosine
  source 1..18: mol_type = other DNA
nnnntgtcaacaagnnnn

SEQ ID NO: 390 - DNA, 17 bp, synthetic construct
  misc_feature 1..17: note = Synthetic Construct
  modified_base 1: mod_base = OTHER; note = locked nucleic acid thymidine
  misc_feature 1..17: note = phosphorothioate backbone
  modified_base 2..3: mod_base = OTHER; note = locked nucleic acid guanosine
  modified_base 14..15: mod_base = OTHER; note = locked nucleic acid 5-methylcytidine
  modified_base 16..17: mod_base = OTHER; note = locked nucleic acid adenosine
  source 1..17: mol_type = other DNA
nnntgtcaacaagnnnn

SEQ ID NO: 391 - DNA, 17 bp, synthetic construct
  misc_feature 1..17: note = Synthetic Construct
  modified_base 1: mod_base = OTHER; note = locked nucleic acid thymidine
  misc_feature 1..3: note = phosphorothioate backbone
  modified_base 2..3: mod_base = OTHER; note = locked nucleic acid guanosine
  misc_feature 3..4: note = phosphodiester backbone
  misc_feature 4..13: note = phosphorothioate backbone
  misc_feature 13..14: note = phosphodiester backbone
  misc_feature 14..17: note = phosphorothioate backbone
  modified_base 14..15: mod_base = OTHER; note = locked nucleic acid 5-methylcytidine
  modified_base 16..17: mod_base = OTHER; note = locked nucleic acid adenosine
  source 1..17: mol_type = other DNA
nnntgtcaacaagnnnn

SEQ ID NO: 392 - DNA, 17 bp, synthetic construct
  misc_feature 1..17: note = Synthetic Construct
  modified_base 1: mod_base = OTHER; note = locked nucleic acid thymidine
  misc_feature 1..2: note = phosphorothioate backbone
  misc_feature 2..3: note = phosphodiester backbone
  modified_base 2..3: mod_base = OTHER; note = locked nucleic acid guanosine
  misc_feature 3..4: note = phosphorothioate backbone
  misc_feature 4..5: note = phosphodiester backbone
  misc_feature 5..6: note = phosphorothioate backbone
  misc_feature 6..7: note = phosphodiester backbone
  misc_feature 7..8: note = phosphorothioate backbone
  misc_feature 8..9: note = phosphodiester backbone
  misc_feature 9..10: note = phosphorothioate backbone
  misc_feature 10..11: note = phosphodiester backbone
  misc_feature 11..12: note = phosphorothioate backbone
  misc_feature 12..13: note = phosphodiester backbone
  misc_feature 13..14: note = phosphorothioate backbone
  misc_feature 14..16: note = phosphodiester backbone
  modified_base 14..15: mod_base = OTHER; note = locked nucleic acid 5-methylcytidine
  misc_feature 16..17: note = phosphorothioate backbone
  modified_base 16..17: mod_base = OTHER; note = locked nucleic acid adenosine
  source 1..17: mol_type = other DNA
nnntgtcaacaagnnnn

SEQ ID NO: 393 - RNA, 20 nt, synthetic construct
  misc_feature 1..20: note = Synthetic Construct
  source 1..20: mol_type = other RNA
gaaaccatctctgggataag

SEQ ID NO: 394 - RNA, 20 nt, synthetic construct
  misc_feature 1..20: note = Synthetic Construct
  source 1..20: mol_type = other RNA
aaaccatctctgggataagg

SEQ ID NO: 395 - RNA, 20 nt, synthetic construct
  misc_feature 1..20: note = Synthetic Construct
  source 1..20: mol_type = other RNA
aaccatctctgggataagga

SEQ ID NO: 396 - RNA, 20 nt, synthetic construct
  misc_feature 1..20: note = Synthetic Construct
  source 1..20: mol_type = other RNA
accatctctgggataaggat

SEQ ID NO: 397 - RNA, 20 nt, synthetic construct
  misc_feature 1..20: note = Synthetic Construct
  source 1..20: mol_type = other RNA
ccatctctgggataaggatg

SEQ ID NO: 398 - RNA, 20 nt, synthetic construct
  misc_feature 1..20: note = Synthetic Construct
  source 1..20: mol_type = other RNA
catctctgggataaggatga

SEQ ID NO: 399 - RNA, 20 nt, synthetic construct
  misc_feature 1..20: note = Synthetic Construct
  source 1..20: mol_type = other RNA
atctctgggataaggatgac

SEQ ID NO: 400 - RNA, 20 nt, synthetic construct
  misc_feature 1..20: note = Synthetic Construct
  source 1..20: mol_type = other RNA
tctctgggataaggatgact

SEQ ID NO: 401 - RNA, 20 nt, synthetic construct
  misc_feature 1..20: note = Synthetic Construct
  source 1..20: mol_type = other RNA
ctctgggataaggatgactg

SEQ ID NO: 402 - RNA, 20 nt, synthetic construct
  misc_feature 1..20: note = Synthetic Construct
  source 1..20: mol_type = other RNA
tctgggataaggatgactga

SEQ ID NO: 403 - RNA, 20 nt, synthetic construct
  misc_feature 1..20: note = Synthetic Construct
  source 1..20: mol_type = other RNA
ctgggataaggatgactgag

SEQ ID NO: 404 - RNA, 20 nt, synthetic construct
  misc_feature 1..20: note = Synthetic Construct
  source 1..20: mol_type = other RNA
tgggataaggatgactgagg

SEQ ID NO: 405 - RNA, 20 nt, synthetic construct
  misc_feature 1..20: note = Synthetic Construct
  source 1..20: mol_type = other RNA
gggataaggatgactgagga

SEQ ID NO: 406 - RNA, 20 nt, synthetic construct
  misc_feature 1..20: note = Synthetic Construct
  source 1..20: mol_type = other RNA
ggataaggatgactgaggaa

SEQ ID NO: 407 - RNA, 20 nt, synthetic construct
  misc_feature 1..20: note = Synthetic Construct
  source 1..20: mol_type = other RNA
gctgaaacaactgaaacttc

SEQ ID NO: 408 - RNA, 20 nt, synthetic construct
  misc_feature 1..20: note = Synthetic Construct
  source 1..20: mol_type = other RNA
gaaacaactgaaacttcagg

SEQ ID NO: 409 - RNA, 20 nt, synthetic construct
  misc_feature 1..20: note = Synthetic Construct
  source 1..20: mol_type = other RNA
aaacaactgaaacttcaggg

SEQ ID NO: 410 - RNA, 20 nt, synthetic construct
  misc_feature 1..20: note = Synthetic Construct
  source 1..20: mol_type = other RNA
aacaactgaaacttcaggga

SEQ ID NO: 411 - RNA, 20 nt, synthetic construct
  misc_feature 1..20: note = Synthetic Construct
  source 1..20: mol_type = other RNA
acaactgaaacttcagggaa

SEQ ID NO: 412 - RNA, 20 nt, synthetic construct
  misc_feature 1..20: note = Synthetic Construct
  source 1..20: mol_type = other RNA
caactgaaacttcagggaaa

SEQ ID NO: 413 - RNA, 20 nt, synthetic construct
  misc_feature 1..20: note = Synthetic Construct
  source 1..20: mol_type = other RNA
actgaaacttcagggaaaag

SEQ ID NO: 414 - RNA, 19 nt, synthetic construct
  misc_feature 1..19: note = Synthetic Construct
  source 1..19: mol_type = other RNA
aaccatctctgggataagg

SEQ ID NO: 415 - RNA, 19 nt, synthetic construct
  misc_feature 1..19: note = Synthetic Construct
  source 1..19: mol_type = other RNA
accatctctgggataagga

SEQ ID NO: 416 - RNA, 19 nt, synthetic construct
  misc_feature 1..19: note = Synthetic Construct
  source 1..19: mol_type = other RNA
ccatctctgggataaggat

SEQ ID NO: 417 - RNA, 19 nt, synthetic construct
  misc_feature 1..19: note = Synthetic Construct
  source 1..19: mol_type = other RNA
catctctgggataaggatg

SEQ ID NO: 418 - RNA, 19 nt, synthetic construct
  misc_feature 1..19: note = Synthetic Construct
  source 1..19: mol_type = other RNA
atctctgggataaggatga

SEQ ID NO: 419 - RNA, 19 nt, synthetic construct
  misc_feature 1..19: note = Synthetic Construct
  source 1..19: mol_type = other RNA
tctctgggataaggatgac

SEQ ID NO: 420 - RNA, 19 nt, synthetic construct
  misc_feature 1..19: note = Synthetic Construct
  source 1..19: mol_type = other RNA
ctctgggataaggatgact

SEQ ID NO: 421 - RNA, 19 nt, synthetic construct
  misc_feature 1..19: note = Synthetic Construct
  source 1..19: mol_type = other RNA
tctgggataaggatgactg

SEQ ID NO: 422 - RNA, 19 nt, synthetic construct
  misc_feature 1..19: note = Synthetic Construct
  source 1..19: mol_type = other RNA
ctgggataaggatgactga

SEQ ID NO: 423 - RNA, 19 nt, synthetic construct
  misc_feature 1..19: note = Synthetic Construct
  source 1..19: mol_type = other RNA
tgggataaggatgactgag

SEQ ID NO: 424 - RNA, 19 nt, synthetic construct
  misc_feature 1..19: note = Synthetic Construct
  source 1..19: mol_type = other RNA
gggataaggatgactgagg

SEQ ID NO: 425 - RNA, 19 nt, synthetic construct
  misc_feature 1..19: note = Synthetic Construct
  source 1..19: mol_type = other RNA
ggataaggatgactgagga

SEQ ID NO: 426 - RNA, 19 nt, synthetic construct
  misc_feature 1..19: note = Synthetic Construct
  source 1..19: mol_type = other RNA
aacaactgaaacttcaggg

SEQ ID NO: 427 - RNA, 19 nt, synthetic construct
  misc_feature 1..19: note = Synthetic Construct
  source 1..19: mol_type = other RNA
acaactgaaacttcaggga

SEQ ID NO: 428 - RNA, 19 nt, synthetic construct
  misc_feature 1..19: note = Synthetic Construct
  source 1..19: mol_type = other RNA
caactgaaacttcagggaa

SEQ ID NO: 429 - RNA, 19 nt, synthetic construct
  misc_feature 1..19: note = Synthetic Construct
  source 1..19: mol_type = other RNA
caactgaaacttcagggaa

SEQ ID NO: 430 - RNA, 18 nt, synthetic construct
  misc_feature 1..18: note = Synthetic Construct
  source 1..18: mol_type = other RNA
ccatctctgggataagga

SEQ ID NO: 431 - RNA, 18 nt, synthetic construct
  misc_feature 1..18: note = Synthetic Construct
  source 1..18: mol_type = other RNA
catctctgggataaggat

SEQ ID NO: 432 - RNA, 18 nt, synthetic construct
  misc_feature 1..18: note = Synthetic Construct
  source 1..18: mol_type = other RNA
atctctgggataaggatg

SEQ ID NO: 433 - RNA, 18 nt, synthetic construct
  misc_feature 1..18: note = Synthetic Construct
  source 1..18: mol_type = other RNA
tctctgggataaggatga

SEQ ID NO: 434 - RNA, 18 nt, synthetic construct
  misc_feature 1..18: note = Synthetic Construct
  source 1..18: mol_type = other RNA
ctctgggataaggatgac

SEQ ID NO: 435 - RNA, 18 nt, synthetic construct
  misc_feature 1..18: note = Synthetic Construct
  source 1..18: mol_type = other RNA
tctgggataaggatgact

SEQ ID NO: 436 - RNA, 18 nt, synthetic construct
  misc_feature 1..18: note = Synthetic Construct
  source 1..18: mol_type = other RNA
ctgggataaggatgactg

SEQ ID NO: 437 - RNA, 18 nt, synthetic construct
  misc_feature 1..18: note = Synthetic Construct
  source 1..18: mol_type = other RNA
tgggataaggatgactga

SEQ ID NO: 438 - RNA, 18 nt, synthetic construct
  misc_feature 1..18: note = Synthetic Construct
  source 1..18: mol_type = other RNA
gggataaggatgactgag

SEQ ID NO: 439 - RNA, 18 nt, synthetic construct
  misc_feature 1..18: note = Synthetic Construct
  source 1..18: mol_type = other RNA
ggataaggatgactgagg

SEQ ID NO: 440 - RNA, 18 nt, synthetic construct
  misc_feature 1..18: note = Synthetic Construct
  source 1..18: mol_type = other RNA
acaactgaaacttcaggg

SEQ ID NO: 441 - DNA, 20 bp, synthetic construct
  misc_feature 1..20: note = Synthetic Construct
  source 1..20: mol_type = other DNA
cttatcccagagatggtttc

SEQ ID NO: 442 - DNA, 20 bp, synthetic construct
  misc_feature 1..20: note = Synthetic Construct
  source 1..20: mol_type = other DNA
ccttatcccagagatggttt

SEQ ID NO: 443 - DNA, 20 bp, synthetic construct
  misc_feature 1..20: note = Synthetic Construct
  source 1..20: mol_type = other DNA
tccttatcccagagatggtt

SEQ ID NO: 444 - DNA, 20 bp, synthetic construct
  misc_feature 1..20: note = Synthetic Construct
  source 1..20: mol_type = other DNA
atccttatcccagagatggt

SEQ ID NO: 445 - DNA, 20 bp, synthetic construct
  misc_feature 1..20: note = Synthetic Construct
  source 1..20: mol_type = other DNA
catccttatcccagagatgg

SEQ ID NO: 446 - DNA, 20 bp, synthetic construct
  misc_feature 1..20: note = Synthetic Construct
  source 1..20: mol_type = other DNA
tcatccttatcccagagatg

SEQ ID NO: 447 - DNA, 20 bp, synthetic construct
  misc_feature 1..20: note = Synthetic Construct
  source 1..20: mol_type = other DNA
gtcatccttatcccagagat

SEQ ID NO: 448 - DNA, 20 bp, synthetic construct
  misc_feature 1..20: note = Synthetic Construct
  source 1..20: mol_type = other DNA
agtcatccttatcccagaga

SEQ ID NO: 449 - DNA, 20 bp, synthetic construct
  misc_feature 1..20: note = Synthetic Construct
  source 1..20: mol_type = other DNA
cagtcatccttatcccagag

SEQ ID NO: 450 - DNA, 20 bp, synthetic construct
  misc_feature 1..20: note = Synthetic Construct
  source 1..20: mol_type = other DNA
tcagtcatccttatcccaga

SEQ ID NO: 451 - DNA, 20 bp, synthetic construct
  misc_feature 1..20: note = Synthetic Construct
  source 1..20: mol_type = other DNA
ctcagtcatccttatcccag

SEQ ID NO: 452 - DNA, 20 bp, synthetic construct
  misc_feature 1..20: note = Synthetic Construct
  source 1..20: mol_type = other DNA
cctcagtcatccttatccca

SEQ ID NO: 453 - DNA, 20 bp, synthetic construct
  misc_feature 1..20: note = Synthetic Construct
  source 1..20: mol_type = other DNA
tcctcagtcatccttatccc

SEQ ID NO: 454 - DNA, 20 bp, synthetic construct
  misc_feature 1..20: note = Synthetic Construct
  source 1..20: mol_type = other DNA
ttcctcagtcatccttatcc

SEQ ID NO: 455 - DNA, 20 bp, synthetic construct
  misc_feature 1..20: note = Synthetic Construct
  source 1..20: mol_type = other DNA
gaagtttcagttgtttcagc

SEQ ID NO: 456 - DNA, 20 bp, synthetic construct
  misc_feature 1..20: note = Synthetic Construct
  source 1..20: mol_type = other DNA
cctgaagtttcagttgtttc

SEQ ID NO: 457 - DNA, 20 bp, synthetic construct
  misc_feature 1..20: note = Synthetic Construct
  source 1..20: mol_type = other DNA
ccctgaagtttcagttgttt

SEQ ID NO: 458 - DNA, 20 bp, synthetic construct
  misc_feature 1..20: note = Synthetic Construct
  source 1..20: mol_type = other DNA
tccctgaagtttcagttgtt

SEQ ID NO: 459 - DNA, 20 bp, synthetic construct
  misc_feature 1..20: note = Synthetic Construct
  source 1..20: mol_type = other DNA
ttccctgaagtttcagttgt

SEQ ID NO: 460 - DNA, 20 bp, synthetic construct
  misc_feature 1..20: note = Synthetic Construct
  source 1..20: mol_type = other DNA
tttccctgaagtttcagttg

SEQ ID NO: 461 - DNA, 20 bp, synthetic construct
  misc_feature 1..20: note = Synthetic Construct
  source 1..20: mol_type = other DNA
cttttccctgaagtttcagt

SEQ ID NO: 462 - DNA, 19 bp, synthetic construct
  misc_feature 1..19: note = Synthetic Construct
  source 1..19: mol_type = other DNA
ccttatcccagagatggtt

SEQ ID NO: 463 - DNA, 19 bp, synthetic construct
  misc_feature 1..19: note = Synthetic Construct
  source 1..19: mol_type = other DNA
tccttatcccagagatggt

SEQ ID NO: 464 - DNA, 19 bp, synthetic construct
  misc_feature 1..19: note = Synthetic Construct
  source 1..19: mol_type = other DNA
atccttatcccagagatgg

SEQ ID NO: 465 - DNA, 19 bp, synthetic construct
  misc_feature 1..19: note = Synthetic Construct
  source 1..19: mol_type = other DNA
catccttatcccagagatg

SEQ ID NO: 466 - DNA, 19 bp, synthetic construct
  misc_feature 1..19: note = Synthetic Construct
  source 1..19: mol_type = other DNA
tcatccttatcccagagat

SEQ ID NO: 467 - DNA, 19 bp, synthetic construct
  misc_feature 1..19: note = Synthetic Construct
  source 1..19: mol_type = other DNA
gtcatccttatcccagaga

SEQ ID NO: 468 - DNA, 19 bp, synthetic construct
  misc_feature 1..19: note = Synthetic Construct
  source 1..19: mol_type = other DNA
agtcatccttatcccagag

SEQ ID NO: 469 - DNA, 19 bp, synthetic construct
  misc_feature 1..19: note = Synthetic Construct
  source 1..19: mol_type = other DNA
cagtcatccttatcccaga

SEQ ID NO: 470 - DNA, 19 bp, synthetic construct
  misc_feature 1..19: note = Synthetic Construct
  source 1..19: mol_type = other DNA
tcagtcatccttatcccag

SEQ ID NO: 471 - DNA, 19 bp, synthetic construct
  misc_feature 1..19: note = Synthetic Construct
  source 1..19: mol_type = other DNA
ctcagtcatccttatccca

SEQ ID NO: 472 - DNA, 19 bp, synthetic construct
  misc_feature 1..19: note = Synthetic Construct
  source 1..19: mol_type = other DNA
cctcagtcatccttatccc

SEQ ID NO: 473 - DNA, 19 bp, synthetic construct
  misc_feature 1..19: note = Synthetic Construct
  source 1..19: mol_type = other DNA
tcctcagtcatccttatcc

SEQ ID NO: 474 - DNA, 19 bp, synthetic construct
  misc_feature 1..19: note = Synthetic Construct
  source 1..19: mol_type = other DNA
ccctgaagtttcagttgtt

SEQ ID NO: 475 - DNA, 19 bp, synthetic construct
  misc_feature 1..19: note = Synthetic Construct
  source 1..19: mol_type = other DNA
tccctgaagtttcagttgt

SEQ ID NO: 476 - DNA, 19 bp, synthetic construct
  misc_feature 1..19: note = Synthetic Construct
  source 1..19: mol_type = other DNA
ttccctgaagtttcagttg

SEQ ID NO: 477 - DNA, 19 bp, synthetic construct
  misc_feature 1..19: note = Synthetic Construct
  source 1..19: mol_type = other DNA
ttccctgaagtttcagttg

SEQ ID NO: 478 - DNA, 18 bp, synthetic construct
  misc_feature 1..18: note = Synthetic Construct
  source 1..18: mol_type = other DNA
tccttatcccagagatgg

SEQ ID NO: 479 - DNA, 18 bp, synthetic construct
  misc_feature 1..18: note = Synthetic Construct
  source 1..18: mol_type = other DNA
atccttatcccagagatg

SEQ ID NO: 480 - DNA, 18 bp, synthetic construct
  misc_feature 1..18: note = Synthetic Construct
  source 1..18: mol_type = other DNA
catccttatcccagagat

SEQ ID NO: 481 - DNA, 18 bp, synthetic construct
  misc_feature 1..18: note = Synthetic Construct
  source 1..18: mol_type = other DNA
tcatccttatcccagaga

SEQ ID NO: 482 - DNA, 18 bp, synthetic construct
  misc_feature 1..18: note = Synthetic Construct
  source 1..18: mol_type = other DNA
gtcatccttatcccagag

SEQ ID NO: 483 - DNA, 18 bp, synthetic construct
  misc_feature 1..18: note = Synthetic Construct
  source 1..18: mol_type = other DNA
agtcatccttatcccaga

SEQ ID NO: 484 - DNA, 18 bp, synthetic construct
  misc_feature 1..18: note = Synthetic Construct
  source 1..18: mol_type = other DNA
cagtcatccttatcccag

SEQ ID NO: 485 - DNA, 18 bp, synthetic construct
  misc_feature 1..18: note = Synthetic Construct
  source 1..18: mol_type = other DNA
tcagtcatccttatccca

SEQ ID NO: 486 - DNA, 18 bp, synthetic construct
  misc_feature 1..18: note = Synthetic Construct
  source 1..18: mol_type = other DNA
ctcagtcatccttatccc

SEQ ID NO: 487 - DNA, 18 bp, synthetic construct
  misc_feature 1..18: note = Synthetic Construct
  source 1..18: mol_type = other DNA
cctcagtcatccttatcc

SEQ ID NO: 488 - DNA, 18 bp, synthetic construct
  misc_feature 1..18: note = Synthetic Construct
  source 1..18: mol_type = other DNA
ccctgaagtttcagttgt

SEQ ID NO: 489 - DNA, 228 bp, synthetic construct
  misc_feature 1..228: note = Synthetic Construct
  source 1..228: mol_type = other DNA
aatgaaatcttctgatttgtaagacatgctgccaagagattagttttacaccttcaggataaagactgctgagaaggtttaaggatgctattctgaaaagactgtggaggaagattaaggaaaccatctctgggataaggatgactgaggaaatttaaggatgccactctggttaaaagctgaaacaactgaaacttcagggaaaagagaaggcctggaatctgatcc

SEQ ID NO: 490 - DNA, 79 bp, synthetic construct
  misc_feature 1..79: note = Synthetic Construct
  source 1..79: mol_type = other DNA
gggtcaatgatgacaacccaatgtcatgaagaaatgtgatgacataaaatttatgctcaataggattacgctgagtccc

SEQ ID NO: 491 - DNA, 79 bp, synthetic construct
  misc_feature 1..79: note = Synthetic Construct
  source 1..79: mol_type = other DNA
gggtcaataatggcaatccaatgtcatgaagaaaggtgatgacataaaattcatgctcaataggattactctgaggccc

SEQ ID NO: 492 - DNA, 88 bp, synthetic construct
  misc_feature 1..88: note = Synthetic Construct
  source 1..88: mol_type = other DNA
gggttcacaaagtgcaatccctcgagccaatgtcatgaagaaaggtgatgacataaaattcatgctcaataggattatgctgaggccc

SEQ ID NO: 493 - DNA, 79 bp, synthetic construct
  misc_feature 1..79: note = Synthetic Construct
  source 1..79: mol_type = other DNA
ttgtcaatgataacaacccaaaatcatgaacagaggtgatgatataaaaatcatgctcaataggattacgctgaggcac

SEQ ID NO: 494 - DNA, 69 bp, synthetic construct
  misc_feature 1..69: note = Synthetic Construct
  source 1..69: mol_type = other DNA
tggccatcataggtcatgaagagtggtgatgacattaaaatcatgatcaataggattacactgaggccc

SEQ ID NO: 495 - DNA, 82 bp, synthetic construct
  misc_feature 1..82: note = Synthetic Construct
  source 1..82: mol_type = other DNA
gggtcaatgatgagaaccttatattgtcctgaagagcggtgatgacttaaaaatcatgctcaataggattacgctgaggccc

SEQ ID NO: 496 - DNA, 76 bp, synthetic construct
  misc_feature 1..76: note = Synthetic Construct
  source 1..76: mol_type = other DNA
gggtcaatgatgagatgttaccttgaagagaaatgatgacgtaaaaattaagttcagttggattacgctgaggccc

SEQ ID NO: 497 - DNA, 53 bp, synthetic construct
  misc_feature 1..53: note = Synthetic Construct
  source 1..53: mol_type = other DNA
ttatattgtcttcgacagggaagatgacataaaaattatgttcaataggatta

SEQ ID NO: 498 - DNA, 71 bp, synthetic construct
  misc_feature 1..71: note = Synthetic Construct
  source 1..71: mol_type = other DNA
tcaataatgaaatcttctgatttggtgagaaataatgccttaaaattacactcaataggattatgctgagg

SEQ ID NO: 499 - DNA, 33 bp, synthetic construct
  misc_feature 1..33: note = Synthetic Construct
  source 1..33: mol_type = other DNA
taaaaatcatgctcaatagaattaagctgaggc

SEQ ID NO: 500 - DNA, 20 bp, synthetic construct
  misc_feature 1..20: note = Synthetic Construct
  source 1..20: mol_type = other DNA
atatgtggaagccggaatct

SEQ ID NO: 501 - DNA, 21 bp, synthetic construct
  misc_feature 1..21: note = Synthetic Construct
  source 1..21: mol_type = other DNA
cccagaactccctaatcagaa

SEQ ID NO: 502 - DNA, 20 bp, synthetic construct
  misc_feature 1..20: note = Synthetic Construct
  source 1..20: mol_type = other DNA
atgacggtggctataccagg

SEQ ID NO: 503 - DNA, 20 bp, synthetic construct
  misc_feature 1..20: note = Synthetic Construct
  source 1..20: mol_type = other DNA
gtctccttcgagctgtttgc

SEQ ID NO: 504 - DNA, 21 bp, synthetic construct
  misc_feature 1..21: note = Synthetic Construct
  source 1..21: mol_type = other DNA
cctttctctccagtgctcaga

SEQ ID NO: 505 - DNA, 21 bp, synthetic construct
  misc_feature 1..21: note = Synthetic Construct
  source 1..21: mol_type = other DNA
cctgtgaactttcaaccagga

SEQ ID NO: 506 - DNA, 20 bp, synthetic construct
  misc_feature 1..20: note = Synthetic Construct
  source 1..20: mol_type = other DNA
ggatcagactccaggccttc

SEQ ID NO: 507 - RNA, 20 nt, synthetic construct
  misc_feature 1..20: note = Synthetic Construct
  source 1..20: mol_type = other RNA
cccaggtgtcctttaatgaa

SEQ ID NO: 508 - RNA, 20 nt, synthetic construct
  misc_feature 1..20: note = Synthetic Construct
  source 1..20: mol_type = other RNA
ccaggtgtcctttaatgaaa

SEQ ID NO: 509 - RNA, 20 nt, synthetic construct
  misc_feature 1..20: note = Synthetic Construct
  source 1..20: mol_type = other RNA
tgaaaatgctcttgacacca

SEQ ID NO: 510 - RNA, 20 nt, synthetic construct
  misc_feature 1..20: note = Synthetic Construct
  source 1..20: mol_type = other RNA
gaaaatgctcttgacaccaa

SEQ ID NO: 511 - RNA, 20 nt, synthetic construct
  misc_feature 1..20: note = Synthetic Construct
  source 1..20: mol_type = other RNA
aaatgctcttgacaccaatg

SEQ ID NO: 512 - RNA, 20 nt, synthetic construct
  misc_feature 1..20: note = Synthetic Construct
  source 1..20: mol_type = other RNA
agatcagtagcttcctttac

SEQ ID NO: 513 - RNA, 20 nt, synthetic construct
  misc_feature 1..20: note = Synthetic Construct
  source 1..20: mol_type = other RNA
tcagtagcttcctttaccga

SEQ ID NO: 514 - RNA, 20 nt, synthetic construct
  misc_feature 1..20: note = Synthetic Construct
  source 1..20: mol_type = other RNA
tctagaacattgagctatgg

SEQ ID NO: 515 - RNA, 20 nt, synthetic construct
  misc_feature 1..20: note = Synthetic Construct
  source 1..20: mol_type = other RNA
ctagaacattgagctatgga

SEQ ID NO: 516 - RNA, 20 nt, synthetic construct
  misc_feature 1..20: note = Synthetic Construct
  source 1..20: mol_type = other RNA
aacattgagctatggaagac

SEQ ID NO: 517 - RNA, 20 nt, synthetic construct
  misc_feature 1..20: note = Synthetic Construct
  source 1..20: mol_type = other RNA
acattgagctatggaagact

SEQ ID NO: 518 - RNA, 20 nt, synthetic construct
  misc_feature 1..20: note = Synthetic Construct
  source 1..20: mol_type = other RNA
ctatggaagactcccaccta

SEQ ID NO: 519 - RNA, 20 nt, synthetic construct
  misc_feature 1..20: note = Synthetic Construct
  source 1..20: mol_type = other RNA
tatggaagactcccacctaa

SEQ ID NO: 520 - RNA, 20 nt, synthetic construct
  misc_feature 1..20: note = Synthetic Construct
  source 1..20: mol_type = other RNA
caagtgctaccgcacaggca

SEQ ID NO: 521 - RNA, 20 nt, synthetic construct
  misc_feature 1..20: note = Synthetic Construct
  source 1..20: mol_type = other RNA
aagtgctaccgcacaggcat

SEQ ID NO: 522 - RNA, 20 nt, synthetic construct
  misc_feature 1..20: note = Synthetic Construct
  source 1..20: mol_type = other RNA
taccgcacaggcatgctgca

SEQ ID NO: 523 - RNA, 20 nt, synthetic construct
  misc_feature 1..20: note = Synthetic Construct
  source 1..20: mol_type = other RNA
caggcatgctgcagtgaatt

SEQ ID NO: 524 - RNA, 20 nt, synthetic construct
  misc_feature 1..20: note = Synthetic Construct
  source 1..20: mol_type = other RNA
aggcatgctgcagtgaattt

SEQ ID NO: 525 - RNA, 20 nt, synthetic construct
  misc_feature 1..20: note = Synthetic Construct
  source 1..20: mol_type = other RNA
accgttgtttaaggatgcta

SEQ ID NO: 526 - RNA, 20 nt, synthetic construct
  misc_feature 1..20: note = Synthetic Construct
  source 1..20: mol_type = other RNA
ccgttgtttaaggatgctat

SEQ ID NO: 527 - RNA, 20 nt, synthetic construct
  misc_feature 1..20: note = Synthetic Construct
  source 1..20: mol_type = other RNA
ctgtggaggaagaaaaccct

SEQ ID NO: 528 - RNA, 20 nt, synthetic construct
  misc_feature 1..20: note = Synthetic Construct
  source 1..20: mol_type = other RNA
aagaaaaccctttaccctgt

SEQ ID NO: 529 - RNA, 20 nt, synthetic construct
  misc_feature 1..20: note = Synthetic Construct
  source 1..20: mol_type = other RNA
agaaaaccctttaccctgtt

SEQ ID NO: 530 - RNA, 20 nt, synthetic construct
  misc_feature 1..20: note = Synthetic Construct
  source 1..20: mol_type = other RNA
ctcaactgcctggcactgaa

SEQ ID NO: 531 - RNA, 20 nt, synthetic construct
  misc_feature 1..20: note = Synthetic Construct
  source 1..20: mol_type = other RNA
aactgcctggcactgaaaat

SEQ ID NO: 532 - RNA, 20 nt, synthetic construct
  misc_feature 1..20: note = Synthetic Construct
  source 1..20: mol_type = other RNA
actgcctggcactgaaaatg

SEQ ID NO: 533 - RNA, 20 nt, synthetic construct
  misc_feature 1..20: note = Synthetic Construct
  source 1..20: mol_type = other RNA
gtgtttaaggaaaccatctc

SEQ ID NO: 534 - RNA, 20 nt, synthetic construct
  misc_feature 1..20: note = Synthetic Construct
  source 1..20: mol_type = other RNA
gtttaaggaaaccatctctg

SEQ ID NO: 535 - RNA, 20 nt, synthetic construct
  misc_feature 1..20: note = Synthetic Construct
  source 1..20: mol_type = other RNA
aggaaaccatctctgataag

SEQ ID NO: 536 - RNA, 20 nt, synthetic construct
  misc_feature 1..20: note = Synthetic Construct
  source 1..20: mol_type = other RNA
tctttggcttgttgacacca

SEQ ID NO: 537 - RNA, 20 nt, synthetic construct
  misc_feature 1..20: note = Synthetic Construct
  source 1..20: mol_type = other RNA
ctttggcttgttgacaccag

SEQ ID NO: 538 - DNA, 20 bp, synthetic construct
  misc_feature 1..20: note = Synthetic Construct
  source 1..20: mol_type = other DNA
ttcattaaaggacacctggg

SEQ ID NO: 539 - DNA, 20 bp, synthetic construct
  misc_feature 1..20: note = Synthetic Construct
  source 1..20: mol_type = other DNA
tttcattaaaggacacctgg

SEQ ID NO: 540 - DNA, 20 bp, synthetic construct
  misc_feature 1..20: note = Synthetic Construct
  source 1..20: mol_type = other DNA
tggtgtcaagagcattttca

SEQ ID NO: 541 - DNA, 20 bp, synthetic construct
  misc_feature 1..20: note = Synthetic Construct
  source 1..20: mol_type = other DNA
ttggtgtcaagagcattttc

SEQ ID NO: 542 - DNA, 20 bp, synthetic construct
  misc_feature 1..20: note = Synthetic Construct
  source 1..20: mol_type = other DNA
cattggtgtcaagagcattt

SEQ ID NO: 543 - DNA, 20 bp, synthetic construct
  misc_feature 1..20: note = Synthetic Construct
  source 1..20: mol_type = other DNA
gtaaaggaagctactgatct

SEQ ID NO: 544 - DNA, 20 bp, synthetic construct
  misc_feature 1..20: note = Synthetic Construct
  source 1..20: mol_type = other DNA
tcggtaaaggaagctactga

SEQ ID NO: 545 - DNA, 20 bp, synthetic construct
  misc_feature 1..20: note = Synthetic Construct
  source 1..20: mol_type = other DNA
ccatagctcaatgttctaga

SEQ ID NO: 546 - DNA, 20 bp, synthetic construct
  misc_feature 1..20: note = Synthetic Construct
  source 1..20: mol_type = other DNA
tccatagctcaatgttctag

SEQ ID NO: 547 - DNA, 20 bp, synthetic construct
  misc_feature 1..20: note = Synthetic Construct
  source 1..20: mol_type = other DNA
gtcttccatagctcaatgtt

SEQ ID NO: 548 - DNA, 20 bp, synthetic construct
  misc_feature 1..20: note = Synthetic Construct
  source 1..20: mol_type = other DNA
agtcttccatagctcaatgt

SEQ ID NO: 549 - DNA, 20 bp, synthetic construct
  misc_feature 1..20: note = Synthetic Construct
  source 1..20: mol_type = other DNA
taggtgggagtcttccatag

SEQ ID NO: 550 - DNA, 20 bp, synthetic construct
  misc_feature 1..20: note = Synthetic Construct
  source 1..20: mol_type = other DNA
ttaggtgggagtcttccata

SEQ ID NO: 551 - DNA, 20 bp, synthetic construct
  misc_feature 1..20: note = Synthetic Construct
  source 1..20: mol_type = other DNA
tgcctgtgcggtagcacttg

SEQ ID NO: 552 - DNA, 20 bp, synthetic construct
  misc_feature 1..20: note = Synthetic Construct
  source 1..20: mol_type = other DNA
atgcctgtgcggtagcactt

SEQ ID NO: 553 - DNA, 20 bp, synthetic construct
  misc_feature 1..20: note = Synthetic Construct
  source 1..20: mol_type = other DNA
tgcagcatgcctgtgcggta

SEQ ID NO: 554 - DNA, 20 bp, synthetic construct
  misc_feature 1..20: note = Synthetic Construct
  source 1..20: mol_type = other DNA
aattcactgcagcatgcctg

SEQ ID NO: 555 - DNA, 20 bp, synthetic construct
  misc_feature 1..20: note = Synthetic Construct
  source 1..20: mol_type = other DNA
aaattcactgcagcatgcct

SEQ ID NO: 556 - DNA, 20 bp, synthetic construct
  misc_feature 1..20: note = Synthetic Construct
  source 1..20: mol_type = other DNA
tagcatccttaaacaacggt

SEQ ID NO: 557 - DNA, 20 bp, synthetic construct
  misc_feature 1..20: note = Synthetic Construct
  source 1..20: mol_type = other DNA
atagcatccttaaacaacgg

SEQ ID NO: 558 - DNA, 20 bp, synthetic construct
  misc_feature 1..20: note = Synthetic Construct
  source 1..20: mol_type = other DNA
agggttttcttcctccacag

SEQ ID NO: 559 - DNA, 20 bp, synthetic construct
  misc_feature 1..20: note = Synthetic Construct
  source 1..20: mol_type = other DNA
acagggtaaagggttttctt

SEQ ID NO: 560 - DNA, 20 bp, synthetic construct
  misc_feature 1..20: note = Synthetic Construct
  source 1..20: mol_type = other DNA
aacagggtaaagggttttct

SEQ ID NO: 561 - DNA, 20 bp, synthetic construct
  misc_feature 1..20: note = Synthetic Construct
  source 1..20: mol_type = other DNA
ttcagtgccaggcagttgag

SEQ ID NO: 562 - DNA, 20 bp, synthetic construct
  misc_feature 1..20: note = Synthetic Construct
  source 1..20: mol_type = other DNA
attttcagtgccaggcagtt

SEQ ID NO: 563 - DNA, 20 bp, synthetic construct
  misc_feature 1..20: note = Synthetic Construct
  source 1..20: mol_type = other DNA
cattttcagtgccaggcagt

SEQ ID NO: 564 - DNA, 20 bp, synthetic construct
  misc_feature 1..20: note = Synthetic Construct
  source 1..20: mol_type = other DNA
gagatggtttccttaaacac

SEQ ID NO: 565 - DNA, 20 bp, synthetic construct
  misc_feature 1..20: note = Synthetic Construct
  source 1..20: mol_type = other DNA
cagagatggtttccttaaac

SEQ ID NO: 566 - DNA, 20 bp, synthetic construct
  misc_feature 1..20: note = Synthetic Construct
  source 1..20: mol_type = other DNA
cttatcagagatggtttcct

SEQ ID NO: 567 - DNA, 20 bp, synthetic construct
  misc_feature 1..20: note = Synthetic Construct
  source 1..20: mol_type = other DNA
tggtgtcaacaagccaaaga

SEQ ID NO: 568 - DNA, 20 bp, synthetic construct
  misc_feature 1..20: note = Synthetic Construct
  source 1..20: mol_type = other DNA
ctggtgtcaacaagccaaag

SEQ ID NO: 569 - DNA, 58 bp, synthetic construct
  misc_feature 1..58: note = Synthetic Construct
  source 1..58: mol_type = other DNA
ggtgccattctattataaataacctgacccattatttataatagaatggcaccttttt

SEQ ID NO: 570 - DNA, 58 bp, synthetic construct
  misc_feature 1..58: note = Synthetic Construct
  source 1..58: mol_type = other DNA
gctttcatcaataatgaaataacctgacccattatttcattattgatgaaagcttttt

SEQ ID NO: 571 - DNA, 58 bp, synthetic construct
  misc_feature 1..58: note = Synthetic Construct
  source 1..58: mol_type = other DNA
ggtctttcatcaataatgataacctgacccattatcattattgatgaaagaccttttt

SEQ ID NO: 572 - DNA, 58 bp, synthetic construct
  misc_feature 1..58: note = Synthetic Construct
  source 1..58: mol_type = other DNA
gaaatcttctgatttgtaataacctgacccattattacaaatcagaagatttcttttt

SEQ ID NO: 573 - DNA, 58 bp, synthetic construct
  misc_feature 1..58: note = Synthetic Construct
  source 1..58: mol_type = other DNA
gcacctaagggaattagtataacctgacccattatactaattcccttaggtgcttttt

SEQ ID NO: 574 - DNA, 58 bp, synthetic construct
  misc_feature 1..58: note = Synthetic Construct
  source 1..58: mol_type = other DNA
gtttcaaccaggatttaaataacctgacccattatttaaatcctggttgaaacttttt

SEQ ID NO: 575 - DNA, 58 bp, synthetic construct
  misc_feature 1..58: note = Synthetic Construct
  source 1..58: mol_type = other DNA
gctttcaaccaggatttaataacctgacccattattaaatcctggttgaaagcttttt

SEQ ID NO: 576 - DNA, 58 bp, synthetic construct
  misc_feature 1..58: note = Synthetic Construct
  source 1..58: mol_type = other DNA
ggagatgtgccattctatataacctgacccattatatagaatggcacatctccttttt

SEQ ID NO: 577 - DNA, 58 bp, synthetic construct
  misc_feature 1..58: note = Synthetic Construct
  source 1..58: mol_type = other DNA
gtctttcatcaataatgaataacctgacccattattcattattgatgaaagacttttt

SEQ ID NO: 578 - DNA, 58 bp, synthetic construct
  misc_feature 1..58: note = Synthetic Construct
  source 1..58: mol_type = other DNA
gatcaataatgaaatcttataacctgacccattataagatttcattattgatcttttt

SEQ ID NO: 579 - DNA, 58 bp, synthetic construct
  misc_feature 1..58: note = Synthetic Construct
  source 1..58: mol_type = other DNA
gtgtctttcatcaataatataacctgacccattatattattgatgaaagacacttttt

SEQ ID NO: 580 - DNA, 58 bp, synthetic construct
  misc_feature 1..58: note = Synthetic Construct
  source 1..58: mol_type = other DNA
gcaataatgaaatcttctataacctgacccattatagaagatttcattattgcttttt

SEQ ID NO: 581 - DNA, 58 bp, synthetic construct
  misc_feature 1..58: note = Synthetic Construct
  source 1..58: mol_type = other DNA
gcatgctgcagtgaatttataacctgacccattataaattcactgcagcatgcttttt

SEQ ID NO: 582 - DNA, 58 bp, synthetic construct
  misc_feature 1..58: note = Synthetic Construct
  source 1..58: mol_type = other DNA
ggaaatcttctgatttgtataacctgacccattatacaaatcagaagatttccttttt

SEQ ID NO: 583 - DNA, 58 bp, synthetic construct
  misc_feature 1..58: note = Synthetic Construct
  source 1..58: mol_type = other DNA
ggtatattctatctagaaataacctgacccattatttctagatagaatataccttttt

SEQ ID NO: 584 - DNA, 58 bp, synthetic construct
  misc_feature 1..58: note = Synthetic Construct
  source 1..58: mol_type = other DNA
gtgctgcagtgaatttaaataacctgacccattatttaaattcactgcagcacttttt

SEQ ID NO: 585 - DNA, 58 bp, synthetic construct
  misc_feature 1..58: note = Synthetic Construct
  source 1..58: mol_type = other DNA
gtgtgccattctattataataacctgacccattattataatagaatggcacacttttt

SEQ ID NO: 586 - DNA, 58 bp, synthetic construct
  misc_feature 1..58: note = Synthetic Construct
  source 1..58: mol_type = other DNA
gttaccatcagtgtttaaataacctgacccattatttaaacactgatggtaacttttt

SEQ ID NO: 587 - DNA, 58 bp, synthetic construct
  misc_feature 1..58: note = Synthetic Construct
  source 1..58: mol_type = other DNA
gcctgcaaccgttgtttaataacctgacccattattaaacaacggttgcaggcttttt

SEQ ID NO: 588 - DNA, 58 bp, synthetic construct
  misc_feature 1..58: note = Synthetic Construct
  source 1..58: mol_type = other DNA
gtatgtctttcatcaataataacctgacccattattattgatgaaagacatacttttt

SEQ ID NO: 589 - DNA, 20 bp, synthetic construct
  misc_feature 1..20: note = Synthetic Construct
  source 1..20: mol_type = other DNA
acactgatggtaaagtggac

SEQ ID NO: 590 - DNA, 20 bp, synthetic construct
  misc_feature 1..20: note = Synthetic Construct
  source 1..20: mol_type = other DNA
tagaatatacacgtcggtaa

SEQ ID NO: 591 - DNA, 20 bp, synthetic construct
  misc_feature 1..20: note = Synthetic Construct
  source 1..20: mol_type = other DNA
tcaactgtcccagtcacaac

SEQ ID NO: 592 - DNA, 20 bp, synthetic construct
  misc_feature 1..20: note = Synthetic Construct
  source 1..20: mol_type = other DNA
tctagatagaatatacacgt

SEQ ID NO: 593 - DNA, 20 bp, synthetic construct
  misc_feature 1..20: note = Synthetic Construct
  source 1..20: mol_type = other DNA
tctagatagaatatacacgt

SEQ ID NO: 594 - DNA, 20 bp, synthetic construct
  misc_feature 1..20: note = Synthetic Construct
  source 1..20: mol_type = other DNA
ctccccatgcacacttgaga

SEQ ID NO: 595 - DNA, 20 bp, synthetic construct
  misc_feature 1..20: note = Synthetic Construct
  source 1..20: mol_type = other DNA
catccttaaacaacggttgc

SEQ ID NO: 596 - DNA, 20 bp, synthetic construct
  misc_feature 1..20: note = Synthetic Construct
  source 1..20: mol_type = other DNA
ggtgtaaaactaattccctt

SEQ ID NO: 597 - DNA, 20 bp, synthetic construct
  misc_feature 1..20: note = Synthetic Construct
  source 1..20: mol_type = other DNA
aacaacggttgcagggacag

SEQ ID NO: 598 - DNA, 20 bp, synthetic construct
  misc_feature 1..20: note = Synthetic Construct
  source 1..20: mol_type = other DNA
tatggaagactcccacctaa

SEQ ID NO: 599 - DNA, 20 bp, synthetic construct
  misc_feature 1..20: note = Synthetic Construct
  source 1..20: mol_type = other DNA
ctatggaagactcccaccta

SEQ ID NO: 600 - DNA, 20 bp, synthetic construct
  misc_feature 1..20: note = Synthetic Construct
  source 1..20: mol_type = other DNA
aagccttctcaagtgtgcat

SEQ ID NO: 601 - DNA, 20 bp, synthetic construct
  misc_feature 1..20: note = Synthetic Construct
  source 1..20: mol_type = other DNA
ctatctagaacattgagcta

SEQ ID NO: 602 - DNA, 20 bp, synthetic construct
  misc_feature 1..20: note = Synthetic Construct
  source 1..20: mol_type = other DNA
accctctggtgttgtcacag

SEQ ID NO: 603 - DNA, 20 bp, synthetic construct
  misc_feature 1..20: note = Synthetic Construct
  source 1..20: mol_type = other DNA
aaccctttaccctgttgttc

SEQ ID NO: 604 - DNA, 79 bp, synthetic construct
  misc_feature 1..79: note = synthetic construct
  modified_base 13: mod_base = OTHER; note = a, c, t, g, unknown or other
  modified_base 17: mod_base = OTHER; note = a, c, t, g, unknown or other
  source 1..79: mol_type = other DNA
gggtcaataatgncaanccaatgtcatgaagaaaggtgatgacataaaattcatgctcaataggattacgctgaggccc

SEQ ID NO: 605 - DNA, 78 bp, synthetic construct
  misc_feature 1..78: note = synthetic construct
  modified_base 20: mod_base = OTHER; note = a, c, t, g, unknown or other
  modified_base 44: mod_base = OTHER; note = a, c, t, g, unknown or other
  source 1..78: mol_type = other DNA
ggtcaatgatgagacttatnttgtcttgaagagagatgatgacntaaaaattatgctcaataggattacgctgaggcc